European Patent Application EP 4 461 745 A1, published November 13, 2024. Title: ANTI-C3b ANTIBODY OR ANTI-C5 ANTIBODY CONJUGATED WITH ANGIOGENESIS INHIBITOR AND USE THEREOF. Applicant: Kanaph Therapeutics Inc. The sequence listing filed with the application follows.

SEQUENCE LISTING (197 sequences)

SEQ ID NO: 1 - protein, 448 aa, synthetic construct
  REGION 1..448: note = anti-C3b (MOR09611) HC
EVQLVESGGGLVQPGGSLRLSCAASGFTFSSYWMTWVRQAPGKGLEWVSSIKIKPDGYAASVKGRFTISRDNSKNTLYLQMNSLRAEDTAVYYCARLFYQYFARMDYWGQGTLVTVSSASTKGPSVFPLAPSSKSTSGGTAALGCLVKDYFPEPVTVSWNSGALTSGVHTFPAVLQSSGLYSLSSVVTVPSSSLGTQTYICNVNHKPSNTKVDKRVEPKSCDKTHTCPPCPAPEAAGGPSVFLFPPKPKDTLMISRTPEVTCVVVDVSHEDPEVKFNWYVDGVEVHNAKTKPREEQYNSTYRVVSVLTVLHQDWLNGKEYKCKVSNKALPAPIEKTISKAKGQPREPQVYTLPPSREEMTKNQVSLTCLVKGFYPSDIAVEWESNGQPENNYKTTPPVLDSDGSFFLYSKLTVDKSRWQQGNVFSCSVMHEALHNHYTQKSLSLSPGK

SEQ ID NO: 2 - protein, 214 aa, synthetic construct
  REGION 1..214: note = anti-C3b (MOR09611) LC
DIQMTQSPSSLSASVGDRVTITCRASQDISNYLNWYQQKPGKAPKLLIYAASNLQSGVPSRFSGSGSGTDFTLTISSLQPEDFATYYCQQHDTFRPTFGQGTKVEIKRTVAAPSVFIFPPSDEQLKSGTASVVCLLNNFYPREAKVQWKVDNALQSGNSQESVTEQDSKDSTYSLSSTLTLSKADYEKHKVYACEVTHQGLSSPVTKSFNRGEC

SEQ ID NO: 3 - protein, 447 aa, synthetic construct
  REGION 1..447: note = anti-C3b (MOR09675) HC
EVQLVQSGAEVKKPGASVKVSCKASGYTFTGYYINWVRQAPGQGLEWMGIISPNQGTTGYAQKFQGRVTMTRDTSISTAYMELSSLRSEDTAVYYCARGNYDHLDYWGQGTLVTVSSASTKGPSVFPLAPSSKSTSGGTAALGCLVKDYFPEPVTVSWNSGALTSGVHTFPAVIQSSGLYSLSSVVTVPSSSLGTQTYICNVNHKPSNTKVDKRVEPKSCDKTHTCPPCPAPEAAGGPSVFLFPPKPKDTLMISRTPEVTCVVVDVSHEDPEVKFNWYVDGVEVHNAKTKPREEQYNSTYRVVSVLTVLHQDWLNGKEYKCKVSNKALPAPIEKTISKAKGQPREPQVYTLPPSREEMTKNQVSLTCLVKGFYPSDIAVEWESNGQPENNYKTTPPVLDSDGSFFLYSKLTVDKSRWQQGNVFSCSVMHEALHNHYTQKSLSLSPGK

SEQ ID NO: 4 - protein, 215 aa, synthetic construct
  REGION 1..215: note = anti-C3b (MOR09675) LC
DIQMTQSPSSLSASVGDRVTITCRASQGISNYLNWYQQKPGKAPKLLIYDASTLQSGVPSRFSGSGSGTDFTLTISSLQPEDFATYYCQQDWHTLPVTFGQGTKVEIKRTVAAPSVFIFPPSDEQLKSGTASVVCLLNNFYPREAKVQWKVDNALQSGNSQESVTEQDSKDSTYSLSSTLTLSKADYEKHKVYACEVTHQGLSSPVTKSFNRGEC

SEQ ID NO: 5 - protein, 453 aa, synthetic construct
  REGION 1..453: note = anti-C3b (S77) HC-hu IgG1 Fc DANG
EVQLVESGGGLVQPGGSLRLSCAASGFSFTSSSVSWVRQAPGKGLEWVGLIYPYNGFNYYADSVKGRFTISADTSKNTAYLQMNSLRAEDTAVYYCARNALYGSGGYYAMDYWGQGTLVTVSSASTKGPSVFPLAPSSKSTSGGTAALGCLVKDYFPEPVTVSWNSGALTSGVHTFPAVIQSSGLYSLSSVVTVPSSSLGTQTYICNVNHKPSNTKVDKRVEPKSCDKTHTCPPCPAPEAAGGPSVFLFPPKPKDTLMISRTPEVTCVVVAVSHEDPEVKFNWYVDGVEVHNAKTKPREEQYGSTYRVVSVLTVLHQDWLNGKEYKCKVSNKALPAPIEKTISKAKGQPREPQVYTLPPSREEMTKNQVSLTCLVKGFYPSDIAVEWESNGQPENNYKTTPPVLDSDGSFFLYSKLTVDKSRWQQGNVFSCSVMHEALHNHYTQKSLSLSPGK

SEQ ID NO: 6 - protein, 214 aa, synthetic construct
  REGION 1..214: note = anti-C3b (S77) LC
DIQMTQSPSSLSASVGDRVTITCRASQDVSTAVAWYQQKPGKAPKLLIYSASFLYSGVPSRFSGSGSGTDFTLTISSLQPEDFATYYCQQSYATLPTFEQGTKVEIKRTVAAPSVFIFPPSDEQLKSGTASVVCLLNNFYPREAKVQWKVDNALQSGNSQESVTEQDSKDSTYSLSSTLTLSKADYEKHKVYACEVTHQGLSSPVTKSFNRGEC

SEQ ID NO: 7 - protein, 452 aa, synthetic construct
  REGION 1..452: note = anti-C5 (Eculizumab) HC-hu IgG1 Fc DANG
QVQLVQSGAEVKKPGASVKVSCKASGYIFSNYWIQWVRQAPGQGLEWMGEILPGSGSTEYTENFKDRVTMTRDTSTSTVYMELSSLRSEDTAVYYCARYFFGSSPNWYFDVWGQGTLVTVSSASTKGPSVFPLAPSSKSTSGGTAALGCLVKDYFPEPVTVSWNSGALTSGVHTFPAVIQSSGLYSLSSVVTVPSSSLGTQTYICNVNHKPSNTKVDKRVEPKSCDKTHTCPPCPAPEAAGGPSVFLFPPKPKDTLMISRTPEVTCVVVAVSHEDPEVKFNWYVDGVEVHNAKTKPREEQYGSTYRVVSVLTVLHQDWLNGKEYKCKVSNKALPAPIEKTISKAKGQPREPQVYTLPPSREEMTKNQVSLTCLVKGFYPSDIAVEWESNGQPENNYKTTPPVLDSDGSFFLYSKLTVDKSRWQQGNVFSCSVMHEALHNHYTQKSLSLSPGK

SEQ ID NO: 8 - protein, 214 aa, synthetic construct [sequence omitted]

SEQ ID NO: 9 - protein, 662 aa, synthetic construct
  REGION 1..662: note = anti-C3b (MOR09611) HC-hu IgG1 Fc DANG-VEGF binder
EVQLVESGGGLVQPGGSLRLSCAASGFTFSSYWMTWVRQAPGKGLEWVSSIKIKPDGYAASVKGRFTISRDNSKNTLYLQMNSLRAEDTAVYYCARLFYQYFARMDYWGQGTLVTVSSASTKGPSVFPLAPSSKSTSGGTAALGCLVKDYFPEPVTVSWNSGALTSGVHTFPAVLQSSGLYSLSSVVTVPSSSLGTQTYICNVNHKPSNTKVDKRVEPKSCDKTHTCPPCPAPEAAGGPSVFLFPPKPKDTLMISRTPEVTCVVVAVSHEDPEVKFNWYVDGVEVHNAKTKPREEQYGSTYRVVSVLTVLHQDWLNGKEYKCKVSNKALPAPIEKTISKAKGQPREPQVYTLPPSREEMTKNQVSLTCLVKGFYPSDIAVEWESNGQPENNYKTTPPVLDSDGSFFLYSKLTVDKSRWQQGNVFSCSVMHEALHNHYTQKSLSLSPGGGGGSGGGGSSDTGRPFVEMYSEIPEIIHMTEGRELVIPCRVTSPNITVTLKKFPLDTLIPDGKRIIWDSRKGFIISNATYKEIGLLTCEATVNGHLYKTNYLTHRQTNTIIDVVLSPSHGIELSVGEKLVLNCTARTELNVGIDFNWEYPSSKHQHKKLVNRDLKTQSGSEMKKFLSTLTIDGVTRSDQGLYTCAASSGLMTKKNSTFVRVHEK

SEQ ID NO: 10 - protein, 661 aa, synthetic construct
  REGION 1..661: note = anti-C3b (MOR09675) HC-hu IgG1 Fc DANG-VEGF binder
EVQLVQSGAEVKKPGASVKVSCKASGYTFTGYYINWVRQAPGQGLEWMGIISPNQGTTGYAQKFQGRVTMTRDTSISTAYMELSSLRSEDTAVYYCARGNYDHLDYWGQGTLVTVSSASTKGPSVFPLAPSSKSTSGGTAALGCLVKDYFPEPVTVSWNSGALTSGVHTFPAVIQSSGLYSLSSVVTVPSSSLGTQTYICNVNHKPSNTKVDKRVEPKSCDKTHTCPPCPAPEAAGGPSVFLFPPKPKDTLMISRTPEVTCVVVAVSHEDPEVKFNWYVDGVEVHNAKTKPREEQYGSTYRVVSVLTVLHQDWLNGKEYKCKVSNKALPAPIEKTISKAKGQPREPQVYTLPPSREEMTKNQVSLTCLVKGFYPSDIAVEWESNGQPENNYKTTPPVLDSDGSFFLYSKLTVDKSRWQQGNVFSCSVMHEALHNHYTQKSLSLSPGGGGGSGGGGSSDTGRPFVEMYSEIPEIIHMTEGRELVIPCRVTSPNITVTLKKFPLDTLIPDGKRIIWDSRKGFIISNATYKEIGLLTCEATVNGHLYKTNYLTHRQTNTIIDVVLSPSHGIELSVGEKLVLNCTARTELNVGIDFNWEYPSSKHQHKKLVNRDLKTQSGSEMKKFLSTLTIDGVTRSDQGLYTCAASSGLMTKKNSTFVRVHEK

SEQ ID NO: 11 - protein, 667 aa, synthetic construct
  REGION 1..667: note = anti-C3b (S77) HC-hu IgG1 Fc DANG-VEGF binder
EVQLVESGGGLVQPGGSLRLSCAASGFSFTSSSVSWVRQAPGKGLEWVGLIYPYNGFNYYADSVKGRFTISADTSKNTAYLQMNSLRAEDTAVYYCARNALYGSGGYYAMDYWGQGTLVTVSSASTKGPSVFPLAPSSKSTSGGTAALGCLVKDYFPEPVTVSWNSGALTSGVHTFPAVIQSSGLYSLSSVVTVPSSSLGTQTYICNVNHKPSNTKVDKRVEPKSCDKTHTCPPCPAPEAAGGPSVFLFPPKPKDTLMISRTPEVTCVVVAVSHEDPEVKFNWYVDGVEVHNAKTKPREEQYGSTYRVVSVLTVLHQDWLNGKEYKCKVSNKALPAPIEKTISKAKGQPREPQVYTLPPSREEMTKNQVSLTCLVKGFYPSDIAVEWESNGQPENNYKTTPPVLDSDGSFFLYSKLTVDKSRWQQGNVFSCSVMHEALHNHYTQKSLSLSPGGGGGSGGGGSSDTGRPFVEMYSEIPEIIHMTEGRELVIPCRVTSPNITVTLKKFPLDTLIPDGKRIIWDSRKGFIISNATYKEIGLLTCEATVNGHLYKTNYLTHRQTNTIIDVVLSPSHGIELSVGEKLVLNCTARTELNVGIDFNWEYPSSKHQHKKLVNRDLKTQSGSEMKKFLSTLTIDGVTRSDQGLYTCAASSGLMTKKNSTFVRVHEK

SEQ ID NO: 12 - protein, 666 aa, synthetic construct
  REGION 1..666: note = anti-C5 (Eculizumab) HC-hu IgG1 Fc DANG-VEGF binder
QVQLVQSGAEVKKPGASVKVSCKASGYIFSNYWIQWVRQAPGQGLEWMGEILPGSGSTEYTENFKDRVTMTRDTSTSTVYMELSSLRSEDTAVYYCARYFFGSSPNWYFDVWGQGTLVTVSSASTKGPSVFPLAPSSKSTSGGTAALGCLVKDYFPEPVTVSWNSGALTSGVHTFPAVIQSSGLYSLSSVVTVPSSSLGTQTYICNVNHKPSNTKVDKRVEPKSCDKTHTCPPCPAPEAAGGPSVFLFPPKPKDTLMISRTPEVTCVVVAVSHEDPEVKFNWYVDGVEVHNAKTKPREEQYGSTYRVVSVLTVLHQDWLNGKEYKCKVSNKALPAPIEKTISKAKGQPREPQVYTLPPSREEMTKNQVSLTCLVKGFYPSDIAVEWESNGQPENNYKTTPPVLDSDGSFFLYSKLTVDKSRWQQGNVFSCSVMHEALHNHYTQKSLSLSPGGGGGSGGGGSSDTGRPFVEMYSEIPEIIHMTEGRELVIPCRVTSPNITVTLKKFPLDTLIPDGKRIIWDSRKGFIISNATYKEIGLLTCEATVNGHLYKTNYLTHRQTNTIIDVVLSPSHGIELSVGEKLVLNCTARTELNVGIDFNWEYPSSKHQHKKLVNRDLKTQSGSEMKKFLSTLTIDGVTRSDQGLYTCAASSGLMTKKNSTFVRVHEK

SEQ ID NO: 13 - protein, 696 aa, synthetic construct
  REGION 1..696: note = VEGF binder-hu IgG1 Fc DANG-anti-C3b (MOR09611) scFv
SDTGRPFVEMYSEIPEIIHMTEGRELVIPCRVTSPNITVTLKKFPLDTLIPDGKRIIWDSRKGFIISNATYKEIGLLTCEATVNGHLYKTNYLTHRQTNTIIDVVLSPSHGIELSVGEKLVLNCTARTELNVGIDFNWEYPSSKHQHKKLVNRDLKTQSGSEMKKFLSTLTIDGVTRSDQGLYTCAASSGLMTKKNSTFVRVHEKGGGGSDKTHTCPPCPAPEAAGGPSVFLFPPKPKDTLMISRTPEVTCVVVAVSHEDPEVKFNWYVDGVEVHNAKTKPREEQYGSTYRVVSVLTVLHQDWLNGKEYKCKVSNKALPAPIEKTISKAKGQPREPQVYTLPPSREEMTKNQVSLTCLVKGFYPSDIAVEWESNGQPENNYKTTPPVLDSDGSFFLYSKLTVDKSRWQQGNVFSCSVMHEALHNHYTQKSLSLSPGGGGGSGGGGSGGGGSEVQLVESGGGLVQPGGSLRLSCAASGFTFSSYWMTWVRQAPGKGLEWVSSIKIKPDGYAASVKGRFTISRDNSKNTLYLQMNSLRAEDTAVYYCARLFYQYFARMDYWGQGTLVTVSSGGGGSGGGGSGGGGSGGGGSDIQMTQSPSSLSASVGDRVTITCRASQDISNYLNWYQQKPGKAPKLLIYAASNLQSGVPSRFSGSGSGTDFTLTISSLQPEDFATYYCQQHDTFRPTFGQGTKVEIK

SEQ ID NO: 14 - protein, 696 aa, synthetic construct
  REGION 1..696: note = VEGF binder-hu IgG1 Fc DANG-anti-C3b (MOR09675) scFv
SDTGRPFVEMYSEIPEIIHMTEGRELVIPCRVTSPNITVTLKKFPLDTLIPDGKRIIWDSRKGFIISNATYKEIGLLTCEATVNGHLYKTNYLTHRQTNTIIDVVLSPSHGIELSVGEKLVLNCTARTELNVGIDFNWEYPSSKHQHKKLVNRDLKTQSGSEMKKFLSTLTIDGVTRSDQGLYTCAASSGLMTKKNSTFVRVHEKGGGGSDKTHTCPPCPAPEAAGGPSVFLFPPKPKDTLMISRTPEVTCVVVAVSHEDPEVKFNWYVDGVEVHNAKTKPREEQYGSTYRVVSVLTVLHQDWLNGKEYKCKVSNKALPAPIEKTISKAKGQPREPQVYTLPPSREEMTKNQVSLTCLVKGFYPSDIAVEWESNGQPENNYKTTPPVLDSDGSFFLYSKLTVDKSRWQQGNVFSCSVMHEALHNHYTQKSLSLSPGGGGGSGGGGSGGGGSEVQLVQSGAEVKKPGASVKVSCKASGYTFTGYYINWVRQAPGQGLEWMGIISPNQGTTGYAQKFQGRVTMTRDTSISTAYMELSSLRSEDTAVYYCARGNYDHLDYWGQGTLVTVSSGGGGSGGGGSGGGGSGGGGSDIQMTQSPSSLSASVGDRVTITCRASQGISNYLNWYQQKPGKAPKLLIYDASTLQSGVPSRFSGSGSGTDFTLTISSLQPEDFATYYCQQDWHTLPVTFGQGTKVEIK

SEQ ID NO: 15 - protein, 701 aa, synthetic construct
  REGION 1..701: note = VEGF binder-hu IgG1 Fc DANG-anti-C3b (S77) scFv
SDTGRPFVEMYSEIPEIIHMTEGRELVIPCRVTSPNITVTLKKFPLDTLIPDGKRIIWDSRKGFIISNATYKEIGLLTCEATVNGHLYKTNYLTHRQTNTIIDVVLSPSHGIELSVGEKLVLNCTARTELNVGIDFNWEYPSSKHQHKKLVNRDLKTQSGSEMKKFLSTLTIDGVTRSDQGLYTCAASSGLMTKKNSTFVRVHEKGGGGSDKTHTCPPCPAPEAAGGPSVFLFPPKPKDTLMISRTPEVTCVVVAVSHEDPEVKFNWYVDGVEVHNAKTKPREEQYGSTYRVVSVLTVLHQDWLNGKEYKCKVSNKALPAPIEKTISKAKGQPREPQVYTLPPSREEMTKNQVSLTCLVKGFYPSDIAVEWESNGQPENNYKTTPPVLDSDGSFFLYSKLTVDKSRWQQGNVFSCSVMHEALHNHYTQKSLSLSPGGGGGSGGGGSGGGGSEVQLVESGGGLVQPGGSLRLSCAASGFSFTSSSVSWVRQAPGKGLEWVGLIYPYNGFNYYADSVKGRFTISADTSKNTAYLQMNSLRAEDTAVYYCARNALYGSGGYYAMDYWGQGTLVTVSSGGGGSGGGGSGGGGSGGGGSDIQMTQSPSSLSASVGDRVTITCRASQDVSTAVAWYQQKPGKAPKLLIYSASFLYSGVPSRFSGSGSGTDFTLTISSLQPEDFATYYCQQSYATLPTFEQGTKVEIK

SEQ ID NO: 16 - protein, 699 aa, synthetic construct
  REGION 1..699: note = VEGF binder-hu IgG1 Fc DANG-anti-C5 (Eculizumab) scFv
SDTGRPFVEMYSEIPEIIHMTEGRELVIPCRVTSPNITVTLKKFPLDTLIPDGKRIIWDSRKGFIISNATYKEIGLLTCEATVNGHLYKTNYLTHRQTNTIIDVVLSPSHGIELSVGEKLVLNCTARTELNVGIDFNWEYPSSKHQHKKLVNRDLKTQSGSEMKKFLSTLTIDGVTRSDQGLYTCAASSGLMTKKNSTFVRVHEKGGGGSDKTHTCPPCPAPEAAGGPSVFLFPPKPKDTLMISRTPEVTCVVVAVSHEDPEVKFNWYVDGVEVHNAKTKPREEQYGSTYRVVSVLTVLHQDWLNGKEYKCKVSNKALPAPIEKTISKAKGQPREPQVYTLPPSREEMTKNQVSLTCLVKGFYPSDIAVEWESNGQPENNYKTTPPVLDSDGSFFLYSKLTVDKSRWQQGNVFSCSVMHEALHNHYTQKSLSLSPGGGGGSGGGGSGGGGSMADIQMTQSPSSLSASVGDRVTITCGASENIYGALNWYQQKPGKAPKLLIYGATNLADGVPSRFSGSGSGTDFTLTISSLQPEDFATYYCQNVLNTPLTFGQGTKVEIKRTGGGGSGGGGSGGGGSQVQLVQSGAEVKKPGASVKVSCKASGYIFSNYWIQWVRQAPGQGLEWMGEILPGSGSTEYTENFKDRVTMTRDTSTSTVYMELSSLRSEDTAVYYCARYFFGSSPNWYFDVWGQGTLVTVSS

SEQ ID NO: 17 - protein, 227 aa, synthetic construct
  REGION 1..227: note = hu IgG1 Fc DANG with Hinge
DKTHTCPPCPAPELLGGPSVFLFPPKPKDTLMISRTPEVTCVVVAVSHEDPEVKFNWYVDGVEVHNAKTKPREEQYGSTYRVVSVLTVLHQDWLNGKEYKCKVSNKALPAPIEKTISKAKGQPREPQVYTLPPSRDELTKNQVSLTCLVKGFYPSDIAVEWESNGQPENNYKTTPPVLDSDGSFFLYSKLTVDKSRWQQGNVFSCSVMHEALHNHYTQKSLSLSPGK

SEQ ID NO: 18 - protein, 710 aa, synthetic construct
  REGION 1..710: note = hu CRIg-hu IgG1 Fc DANG-VEGF binder
RPILEVPESVTGPWKGDVNLPCTYDPLQGYTQVLVKWLVQRGSDPVTIFLRDSSGDHIQQAKYQGRLHVSHKVPGDVSLQLSTLEMDDRSHYTCEVTWQTPDGNQVVRDKITELRVQKLSVSKPTVTTGSGYGFTVPQGMRISLQCQARGSPPISYIWYKQQTNNQEPIKVATLSTLLFKPAVIADSGSYFCTAKGQVGSEQHSDIVKFVVKDSSKLLKTKTEAPTTMTYPLKATSTVKQSWDWTTDMDGYLGETSAGPGKSLPGGGGSDKTHTCPPCPAPELLGGPSVFLFPPKPKDTLMISRTPEVTCVVVAVSHEDPEVKFNWYVDGVEVHNAKTKPREEQYGSTYRVVSVLTVLHQDWLNGKEYKCKVSNKALPAPIEKTISKAKGQPREPQVYTLPPSRDELTKNQVSLTCLVKGFYPSDIAVEWESNGQPENNYKTTPPVLDSDGSFFLYSKLTVDKSRWQQGNVFSCSVMHEALHNHYTQKSLSLSPGGGGGSGGGGSSDTGRPFVEMYSEIPEIIHMTEGRELVIPCRVTSPNITVTLKKFPLDTLIPDGKRIIWDSRKGFIISNATYKEIGLLTCEATVNGHLYKTNYLTHRQTNTIIDVVLSPSHGIELSVGEKLVLNCTARTELNVGIDFNWEYPSSKHQHKKLVNRDLKTQSGSEMKKFLSTLTIDGVTRSDQGLYTCAASSGLMTKKNSTFVRVHEK

SEQ ID NO: 19 - protein, 432 aa, synthetic construct
  REGION 1..432: note = VEGF binder-hu IgG1 Fc
SDTGRPFVEMYSEIPEIIHMTEGRELVIPCRVTSPNITVTLKKFPLDTLIPDGKRIIWDSRKGFIISNATYKEIGLLTCEATVNGHLYKTNYLTHRQTNTIIDVVLSPSHGIELSVGEKLVLNCTARTELNVGIDFNWEYPSSKHQHKKLVNRDLKTQSGSEMKKFLSTLTIDGVTRSDQGLYTCAASSGLMTKKNSTFVRVHEKDKTHTCPPCPAPELLGGPSVFLFPPKPKDTLMISRTPEVTCVVVDVSHEDPEVKFNWYVDGVEVHNAKTKPREEQYNSTYRVVSVLTVLHQDWLNGKEYKCKVSNKALPAPIEKTISKAKGQPREPQVYTLPPSRDELTKNQVSLTCLVKGFYPSDIAVEWESNGQPENNYKTTPPVLDSDGSFFLYSKLTVDKSRWQQGNVFSCSVMHEALHNHYTQKSLSLSPGK

SEQ ID NO: 20 - protein, 5 aa, synthetic construct
  REGION 1..5: note = anti-C3b HCDR1 (MOR09611)
SYWMT

SEQ ID NO: 21 - protein, 15 aa, synthetic construct
  REGION 1..15: note = anti-C3b HCDR2 (MOR09611)
SIKIKPDGYAASVKG

SEQ ID NO: 22 - protein, 11 aa, synthetic construct
  REGION 1..11: note = anti-C3b HCDR3 (MOR09611)
LFYQYFARMDY

SEQ ID NO: 23 - protein, 11 aa, synthetic construct
  REGION 1..11: note = anti-C3b LCDR1 (MOR09611)
RASQDISNYLN

SEQ ID NO: 24 - protein, 7 aa, synthetic construct
  REGION 1..7: note = anti-C3b LCDR2 (MOR09611)
AASNLQS

SEQ ID NO: 25 - protein, 9 aa, synthetic construct
  REGION 1..9: note = anti-C3b LCDR3 (MOR09611)
QQHDTFRPT

SEQ ID NO: 26 - protein, 118 aa, synthetic construct
  REGION 1..118: note = anti-C3b VH (MOR09611)
EVQLVESGGGLVQPGGSLRLSCAASGFTFSSYWMTWVRQAPGKGLEWVSSIKIKPDGYAASVKGRFTISRDNSKNTLYLQMNSLRAEDTAVYYCARLFYQYFARMDYWGQGTLVTVSS

SEQ ID NO: 27 - protein, 107 aa, synthetic construct
  REGION 1..107: note = anti-C3b VL (MOR09611)
DIQMTQSPSSLSASVGDRVTITCRASQDISNYLNWYQQKPGKAPKLLIYAASNLQSGVPSRFSGSGSGTDFTLTISSLQPEDFATYYCQQHDTFRPTFGQGTKVEIK

SEQ ID NO: 28 - protein, 5 aa, synthetic construct
  REGION 1..5: note = anti-C3b HCDR1 (MOR09675)
GYYIN

SEQ ID NO: 29 - protein, 17 aa, synthetic construct
  REGION 1..17: note = anti-C3b HCDR2 (MOR09675)
IISPNQGTTGYAQKFQG

SEQ ID NO: 30 - protein, 8 aa, synthetic construct
  REGION 1..8: note = anti-C3b HCDR3 (MOR09675)
GNYDHLDY

SEQ ID NO: 31 - protein, 11 aa, synthetic construct
  REGION 1..11: note = anti-C3b LCDR1 (MOR09675)
RASQGISNYLN

SEQ ID NO: 32 - protein, 7 aa, synthetic construct
  REGION 1..7: note = anti-C3b LCDR2 (MOR09675)
DASTLQS

SEQ ID NO: 33 - protein, 10 aa, synthetic construct
  REGION 1..10: note = anti-C3b LCDR3 (MOR09675)
QQDWHTLPVT

SEQ ID NO: 34 - protein, 117 aa, synthetic construct
  REGION 1..117: note = anti-C3b VH (MOR09675)
EVQLVQSGAEVKKPGASVKVSCKASGYTFTGYYINWVRQAPGQGLEWMGIISPNQGTTGYAQKFQGRVTMTRDTSISTAYMELSSLRSEDTAVYYCARGNYDHLDYWGQGTLVTVSS

SEQ ID NO: 35 - protein, 108 aa, synthetic construct
  REGION 1..108: note = anti-C3b VL (MOR09675)
DIQMTQSPSSLSASVGDRVTITCRASQGISNYLNWYQQKPGKAPKLLIYDASTLQSGVPSRFSGSGSGTDFTLTISSLQPEDFATYYCQQDWHTLPVTFGQGTKVEIK

SEQ ID NO: 36 - protein, 10 aa, synthetic construct
  REGION 1..10: note = anti-C3b (S77) HCDR1
GFSFTSSSVS

SEQ ID NO: 37 - protein, 17 aa, synthetic construct
  REGION 1..17: note = anti-C3b (S77) HCDR2
LIYPYNGFNYYADSVKG

SEQ ID NO: 38 - protein, 14 aa, synthetic construct
  REGION 1..14: note = anti-C3b (S77) HCDR3
NALYGSGGYYAMDY

SEQ ID NO: 39 - protein, 11 aa, synthetic construct
  REGION 1..11: note = anti-C3b (S77) LCDR1
RASQDVSTAVA

SEQ ID NO: 40 - protein, 7 aa, synthetic construct
  REGION 1..7: note = anti-C3b (S77) LCDR2
SASFLYS

SEQ ID NO: 41 - protein, 9 aa, synthetic construct
  REGION 1..9: note = anti-C3b (S77) LCDR3
QQSYATLPT

SEQ ID NO: 42 - protein, 123 aa, synthetic construct
  REGION 1..123: note = anti-C3b (S77) VH
EVQLVESGGGLVQPGGSLRLSCAASGFSFTSSSVSWVRQAPGKGLEWVGLIYPYNGFNYYADSVKGRFTISADTSKNTAYLQMNSLRAEDTAVYYCARNALYGSGGYYAMDYWGQGTLVTVSS

SEQ ID NO: 43 - protein, 107 aa, synthetic construct
  REGION 1..107: note = anti-C3b (S77) VL
DIQMTQSPSSLSASVGDRVTITCRASQDVSTAVAWYQQKPGKAPKLLIYSASFLYSGVPSRFSGSGSGTDFTLTISSLQPEDFATYYCQQSYATLPTFEQGTKVEIK

SEQ ID NO: 44 - protein, 5 aa, synthetic construct
  REGION 1..5: note = anti-C5 (Eculizumab) HCDR1
NYWIQ

SEQ ID NO: 45 - protein, 17 aa, synthetic construct
  REGION 1..17: note = anti-C5 (Eculizumab) HCDR2
EILPGSGSTEYTENFKD

SEQ ID NO: 46 - protein, 13 aa, synthetic construct
  REGION 1..13: note = anti-C5 (Eculizumab) HCDR3
YFFGSSPNWYFDV

SEQ ID NO: 47 - protein, 11 aa, synthetic construct
  REGION 1..11: note = anti-C5 (Eculizumab) LCDR1
GASENIYGALN

SEQ ID NO: 48 - protein, 7 aa, synthetic construct
  REGION 1..7: note = anti-C5 (Eculizumab) LCDR2
GATNLAD

SEQ ID NO: 49 - protein, 9 aa, synthetic construct
  REGION 1..9: note = anti-C5 (Eculizumab) LCDR3
QNVLNTPLT

SEQ ID NO: 50 - protein, 122 aa, synthetic construct [sequence omitted]

SEQ ID NO: 51 - protein, 107 aa, synthetic construct [sequence omitted]

SEQ ID NO: 52 - protein, 205 aa, synthetic construct
  REGION 1..205: note = VEGF binder (VEGFR1 D2-VEGFR2 D3)
SDTGRPFVEMYSEIPEIIHMTEGRELVIPCRVTSPNITVTLKKFPLDTLIPDGKRIIWDSRKGFIISNATYKEIGLLTCEATVNGHLYKTNYLTHRQTNTIIDVVLSPSHGIELSVGEKLVLNCTARTELNVGIDFNWEYPSSKHQHKKLVNRDLKTQSGSEMKKFLSTLTIDGVTRSDQGLYTCAASSGLMTKKNSTFVRVHEK

SEQ ID NO: 53 - protein, 23 aa, synthetic construct
  REGION 1..23: note = Linker 1
EPKSCDKTHTCPPCPAPEAAGGP

SEQ ID NO: 54 - protein, 18 aa, synthetic construct
  REGION 1..18: note = Linker 2
DKTHTCPPCPAPELLGGP

SEQ ID NO: 55 - protein, 18 aa, synthetic construct
  REGION 1..18: note = Linker 3
DKTHTCPPCPAPEAAGGP

SEQ ID NO: 56 - protein, 23 aa, synthetic construct
  REGION 1..23: note = Linker 4
GGGGSDKTHTCPPCPAPEAAGGP

SEQ ID NO: 57 - protein, 23 aa, synthetic construct
  REGION 1..23: note = Linker 5
GGGGSDKTHTCPPCPAPELLGGP

SEQ ID NO: 58 - protein, 5 aa, synthetic construct
  REGION 1..5: note = Linker 6
GGGGS

SEQ ID NO: 59 - protein, 10 aa, synthetic construct
  REGION 1..10: note = Linker 7
GGGGSGGGGS

SEQ ID NO: 60 - protein, 15 aa, synthetic construct
  REGION 1..15: note = Linker 8
GGGGSGGGGSGGGGS

SEQ ID NO: 61 - protein, 20 aa, synthetic construct
  REGION 1..20: note = Linker 9
GGGGSGGGGSGGGGSGGGGS

SEQ ID NO: 62 - protein, 208 aa, synthetic construct
  REGION 1..208: note = Human IgG1 Fc DANG (AG-DL)
SVFLFPPKPKDTLMISRTPEVTCVVVAVSHEDPEVKFNWYVDGVEVHNAKTKPREEQYGSTYRVVSVLTVLHQDWLNGKEYKCKVSNKALPAPIEKTISKAKGQPREPQVYTLPPSRDELTKNQVSLTCLVKGFYPSDIAVEWESNGQPENNYKTTPPVLDSDGSFFLYSKLTVDKSRWQQGNVFSCSVMHEALHNHYTQKSLSLSPG

SEQ ID NO: 63 - protein, 208 aa, synthetic construct
  REGION 1..208: note = Human IgG1 Fc DANG (AG-EM)
SVFLFPPKPKDTLMISRTPEVTCVVVAVSHEDPEVKFNWYVDGVEVHNAKTKPREEQYGSTYRVVSVLTVLHQDWLNGKEYKCKVSNKALPAPIEKTISKAKGQPREPQVYTLPPSREEMTKNQVSLTCLVKGFYPSDIAVEWESNGQPENNYKTTPPVLDSDGSFFLYSKLTVDKSRWQQGNVFSCSVMHEALHNHYTQKSLSLSPG

SEQ ID NO: 64 - protein, 209 aa, synthetic construct
  REGION 1..209: note = Human IgG1 Fc DANG-K (AG-DL)
SVFLFPPKPKDTLMISRTPEVTCVVVAVSHEDPEVKFNWYVDGVEVHNAKTKPREEQYGSTYRVVSVLTVLHQDWLNGKEYKCKVSNKALPAPIEKTISKAKGQPREPQVYTLPPSRDELTKNQVSLTCLVKGFYPSDIAVEWESNGQPENNYKTTPPVLDSDGSFFLYSKLTVDKSRWQQGNVFSCSVMHEALHNHYTQKSLSLSPGK

SEQ ID NO: 65 - protein, 209 aa, synthetic construct
  REGION 1..209: note = Human IgG1 Fc-K (DN-DL)
SVFLFPPKPKDTLMISRTPEVTCVVVDVSHEDPEVKFNWYVDGVEVHNAKTKPREEQYNSTYRVVSVLTVLHQDWLNGKEYKCKVSNKALPAPIEKTISKAKGQPREPQVYTLPPSRDELTKNQVSLTCLVKGFYPSDIAVEWESNGQPENNYKTTPPVLDSDGSFFLYSKLTVDKSRWQQGNVFSCSVMHEALHNHYTQKSLSLSPGK

SEQ ID NO: 66 - protein, 209 aa, synthetic construct
  REGION 1..209: note = Human IgG1 Fc DANG-K (AG-EM)
SVFLFPPKPKDTLMISRTPEVTCVVVAVSHEDPEVKFNWYVDGVEVHNAKTKPREEQYGSTYRVVSVLTVLHQDWLNGKEYKCKVSNKALPAPIEKTISKAKGQPREPQVYTLPPSREEMTKNQVSLTCLVKGFYPSDIAVEWESNGQPENNYKTTPPVLDSDGSFFLYSKLTVDKSRWQQGNVFSCSVMHEALHNHYTQKSLSLSPGK

SEQ ID NO: 67 - protein, 209 aa, synthetic construct
  REGION 1..209: note = Human IgG1 Fc-K (DN-EM)
SVFLFPPKPKDTLMISRTPEVTCVVVDVSHEDPEVKFNWYVDGVEVHNAKTKPREEQYNSTYRVVSVLTVLHQDWLNGKEYKCKVSNKALPAPIEKTISKAKGQPREPQVYTLPPSREEMTKNQVSLTCLVKGFYPSDIAVEWESNGQPENNYKTTPPVLDSDGSFFLYSKLTVDKSRWQQGNVFSCSVMHEALHNHYTQKSLSLSPGK

SEQ ID NO: 68 - protein, 208 aa, synthetic construct
  REGION 1..208: note = Human IgG1 Fc WT
SVFLFPPKPKDTLMISRTPEVTCVVVDVSHEDPEVKFNWYVDGVEVHNAKTKPREEQYNSTYRVVSVLTVLHQDWLNGKEYKCKVSNKALPAPIEKTISKAKGQPREPQVYTLPPSRDELTKNQVSLTCLVKGFYPSDIAVEWESNGQPENNYKTTPPVLDSDGSFFLYSKLTVDKSRWQQGNVFSCSVMHEALHNHYTQKSLSLSPG

SEQ ID NO: 69 - DNA, 1347 bp, synthetic construct
  misc_feature 1..1347: note = anti-C3b HC (MOR09611)
  source 1..1347: mol_type = other DNA
gaggtgcagctggtggagagcggcggcggactggtgcagcctggaggatctctgcggctgagctgtgccgctagcggctttaccttcagctcctattggatgacctgggtgaggcaggctcctggcaagggcctggagtgggtgtccagcatcaagatcaagcctgatggctatgctgctagcgtgaagggccggttcaccatctccagggacaacagcaagaacaccctgtacctgcagatgaatagcctgcgggccgaggataccgctgtgtactactgcgccaggctgttctatcagtacttcgctaggatggactattggggccagggcaccctggtgaccgtgagcagcgctagcaccaagggcccctccgtgtttcccctggcccctagctccaagagcaccagcggcggcaccgccgctctgggatgtctggtgaaggactattttcctgagcctgtgaccgtgtcctggaacagcggcgccctgaccagcggcgtgcacacattccccgctgtgctgcagagctccggcctgtactccctgagctccgtggtgaccgtgcctagctccagcctgggcacccagacctacatctgcaatgtgaaccacaagccctccaacaccaaggtggacaagagggtggagcctaagagctgcgacaagacccacacctgccctccttgccccgccccagaggctgctggaggaccttccgtgtttctgttcccccctaagcccaaggataccctgatgatctcccggacccccgaggtgacctgtgtggtggtggacgtgtcccacgaggaccctgaggtgaagtttaactggtacgtggacggcgtggaggtgcacaacgccaagaccaagcccagggaggagcagtacaactccacctacagggtggtgtccgtgctgaccgtgctgcaccaggactggctgaacggcaaggagtataagtgtaaggtgtccaataaggccctgcctgcccccatcgagaagaccatctccaaggccaagggccagcctcgggagcctcaggtgtataccctgcctccctccagggaggagatgaccaagaatcaggtgtccctgacctgtctggtgaaaggcttctatcccagcgacatcgccgtggagtgggagagcaacggccagcccgagaacaactataagaccaccccccctgtgctggacagcgacggctccttctttctgtacagcaagctgaccgtggataagagcaggtggcagcagggcaacgtgttcagctgcagcgtgatgcacgaggctctgcacaaccactatacccagaagagcctgagcctgtcccctggcaagtga

SEQ ID NO: 70 - DNA, 645 bp, synthetic construct
  misc_feature 1..645: note = anti-C3b LC (MOR09611)
  source 1..645: mol_type = other DNA
gacatccagatgacccagagccccagcagcctgagcgccagcgtgggagatcgggtgaccatcacctgtagggccagccaggatatcagcaattatctgaattggtaccagcagaagcccggcaaggctcccaagctgctgatctacgccgcttccaatctgcagtccggcgtgcccagcaggttcagcggctccggaagcggcaccgactttaccctgaccatctccagcctgcagcccgaggattttgctacctactactgccagcagcacgacaccttcaggcctaccttcggccagggcaccaaggtggagatcaagaggacagtggccgctccaagcgtgttcatctttccaccctctgacgagcagctgaagtctggcaccgcttccgtggtgtgcctgctgaacaatttctacccccgggaggctaaggtgcagtggaaggtggataacgccctgcagtccggcaatagccaggagtctgtgaccgagcaggactccaaggatagcacatattctctgagctctaccctgacactgtccaaggctgattacgagaagcacaaggtgtatgcctgcgaggtgacccatcagggcctgtccagccctgtgacaaagagctttaatcgcggcgagtgttga

SEQ ID NO: 71 - DNA, 1344 bp, synthetic construct
  misc_feature 1..1344: note = anti-C3b HC (MOR09675)
  source 1..1344: mol_type = other DNA
gaggtgcagctggtgcagtccggcgccgaggtgaagaagcctggcgctagcgtgaaggtgtcctgcaaggcttccggctacaccttcaccggctactatatcaactgggtgaggcaggctcctggccagggcctggagtggatgggcatcatcagccctaaccagggcaccaccggctacgcccagaagttccagggcagggtgaccatgaccagggacaccagcatcagcaccgcctacatggagctgtccagcctgcggtccgaggacaccgccgtgtactattgtgccaggggcaactacgatcacctggactattggggccagggcaccctggtgaccgtgagctccgctagcaccaagggcccctccgtgtttcccctggcccctagctccaagagcaccagcggcggcaccgccgctctgggatgtctggtgaaggactattttcctgagcctgtgaccgtgtcctggaacagcggcgccctgaccagcggcgtgcacacattccccgctgtgatccagagctccggcctgtactccctgagctccgtggtgaccgtgcctagctccagcctgggcacccagacctacatctgcaatgtgaaccacaagccctccaacaccaaggtggacaagagggtggagcctaagagctgcgacaagacccacacctgccctccttgccccgccccagaggctgctggaggaccttccgtgtttctgttcccccctaagcccaaggataccctgatgatctcccggacccccgaggtgacctgtgtggtggtggacgtgtcccacgaggaccctgaggtgaagtttaactggtacgtggacggcgtggaggtgcacaacgccaagaccaagcccagggaggagcagtacaactccacctacagggtggtgtccgtgctgaccgtgctgcaccaggactggctgaacggcaaggagtataagtgtaaggtgtccaataaggccctgcctgcccccatcgagaagaccatctccaaggccaagggccagcctcgggagcctcaggtgtataccctgcctccctccagggaggagatgaccaagaatcaggtgtccctgacctgtctggtgaaaggcttctatcccagcgacatcgccgtggagtgggagagcaacggccagcccgagaacaactataagaccaccccccctgtgctggacagcgacggctccttctttctgtacagcaagctgaccgtggataagagcaggtggcagcagggcaacgtgttcagctgcagcgtgatgcacgaggctctgcacaaccactatacccagaagagcctgagcctgtcccctggcaagtga

SEQ ID NO: 72 - DNA, 648 bp, synthetic construct
  misc_feature 1..648: note = anti-C3b LC (MOR09675)
  source 1..648: mol_type = other DNA
gatatccagatgacccagtcccccagcagcctgagcgcctccgtgggagatcgggtgaccatcacctgtagggcctcccagggcatcagcaactatctgaattggtaccagcagaagcccggcaaggctcccaagctgctgatctacgacgctagcaccctgcagtccggcgtgccctccagattcagcggcagcggctccggcaccgacttcaccctgaccatcagctccctgcagcctgaggatttcgccacctactattgtcagcaggactggcacaccctgcctgtgaccttcggccagggcaccaaggtggagatcaagaggacagtggccgctccaagcgtgttcatctttccaccctctgacgagcagctgaagtctggcaccgcttccgtggtgtgcctgctgaacaatttctacccccgggaggctaaggtgcagtggaaggtggataacgccctgcagtccggcaatagccaggagtctgtgaccgagcaggactccaaggatagcacatattctctgagctctaccctgacactgtccaaggctgattacgagaagcacaaggtgtatgcctgcgaggtgacccatcagggcctgtccagccctgtgacaaagagctttaatcgcggcgagtgttga

SEQ ID NO: 73 - DNA, 1362 bp, synthetic construct
  misc_feature 1..1362: note = anti-C3b (S77) HC-hu IgG1 Fc DANG
  source 1..1362: mol_type = other DNA
gaagtgcagctggttgagagcggcggaggcctcgtgcaacctggcggatctctgcggctgtcttgtgctgcttctggcttcagcttcacctccagcagcgtgtcctgggtgcggcaggcccctggaaaaggcctggaatgggtcggcctgatctacccctacaacggctttaactactacgccgacagcgtgaagggcagattcaccatcagcgccgataccagcaagaacaccgcctacctgcagatgaacagcctgagagccgaggacacagccgtgtactactgcgccagaaatgccctgtacggcagcggcggatattacgccatggactactggggccagggcaccctggtgacagtgtccagcgctagcaccaagggcccctccgtgtttcccctggcccctagctccaagagcaccagcggcggcaccgccgctctgggatgtctggtgaaggactattttcctgagcctgtgaccgtgtcctggaacagcggcgccctgaccagcggcgtgcacacattccccgctgtgatccagagctccggcctgtactccctgagctccgtggtgaccgtgcctagctccagcctgggcacccagacctacatctgcaatgtgaaccacaagccctccaacaccaaggtggacaagagggtggagcctaagagctgcgacaagacccacacctgccctccttgccccgccccagaggctgctggaggaccttccgtgtttctgttcccccctaagcccaaggataccctgatgatctcccggacccccgaggtgacctgtgtggtggtggctgtgtcccacgaggaccctgaggtgaagtttaactggtacgtggacggcgtggaggtgcacaacgccaagaccaagcccagggaggagcagtacggctccacctacagggtggtgtccgtgctgaccgtgctgcaccaggactggctgaacggcaaggagtataagtgtaaggtgtccaataaggccctgcctgcccccatcgagaagaccatctccaaggccaagggccagcctcgggagcctcaggtgtataccctgcctccctccagggaggagatgaccaagaatcaggtgtccctgacctgtctggtgaaaggcttctatcccagcgacatcgccgtggagtgggagagcaacggccagcccgagaacaactataagaccaccccccctgtgctggacagcgacggctccttctttctgtacagcaagctgaccgtggataagagcaggtggcagcagggcaacgtgttcagctgcagcgtgatgcacgaggctctgcacaaccactatacccagaagagcctgagcctgtcccctggcaagtga

SEQ ID NO: 74 - DNA, 645 bp, synthetic construct
  misc_feature 1..645: note = anti-C3b (S77) LC
  source 1..645: mol_type = other DNA
gatatccagatgacacagagcccaagcagcctgagcgcttctgtgggcgaccgggtgaccatcacatgtagagccagccaggacgtgtccaccgccgtggcctggtaccagcagaaacccggcaaggcccctaagctgctgatctactccgctagcttcctgtacagcggcgtccccagcagattcagcggatctggcagcggcacagattttaccctgaccatcagctccctgcagcctgaggacttcgccacctactactgccagcaatcttatgccacactgcctaccttcgagcagggcaccaaggtggaaatcaagaggacagtggccgccccttccgtgttcatctttccaccctctgacgagcagctgaagtctggcaccgccagcgtggtgtgcctgctgaacaacttctacccacgcgaggccaaggtgcagtggaaggtggataacgccctgcagagcggcaattcccaggagtctgtgacagagcaggacagcaaggattccacctattctctgtctagcaccctgacactgagcaaggccgattacgagaagcacaaggtgtatgcctgcgaggtgacacaccagggcctgtcctctcccgtgaccaagtccttcaacaggggcgagtgttga

SEQ ID NO: 75 - DNA, 1359 bp, synthetic construct
  misc_feature 1..1359: note = anti-C5 (Eculizumab) HC-hu IgG1 Fc DANG
  source 1..1359: mol_type = other DNA
caggtgcagctggtgcagagcggcgccgaggtgaagaaacccggagctagcgtgaaggtgtcttgtaaggcctctggctacatcttcagcaattactggatccagtgggtcagacaggcccctggccagggcctggaatggatgggcgagatcctgcctggaagcggctctaccgagtacaccgaaaacttcaaggacagagtgaccatgacccgggataccagcacaagcaccgtttacatggaactgagctccctgcggagcgaggacacagccgtgtattactgcgccagatactttttcggcagctccccaaactggtacttcgacgtgtggggccaaggcaccctggtgacagtgtccagcgctagcaccaagggcccctccgtgtttcccctggcccctagctccaagagcaccagcggcggcaccgccgctctgggatgtctggtgaaggactattttcctgagcctgtgaccgtgtcctggaacagcggcgccctgaccagcggcgtgcacacattccccgctgtgatccagagctccggcctgtactccctgagctccgtggtgaccgtgcctagctccagcctgggcacccagacctacatctgcaatgtgaaccacaagccctccaacaccaaggtggacaagagggtggagcctaagagctgcgacaagacccacacctgccctccttgccccgccccagaggctgctggaggaccttccgtgtttctgttcccccctaagcccaaggataccctgatgatctcccggacccccgaggtgacctgtgtggtggtggctgtgtcccacgaggaccctgaggtgaagtttaactggtacgtggacggcgtggaggtgcacaacgccaagaccaagcccagggaggagcagtacggctccacctacagggtggtgtccgtgctgaccgtgctgcaccaggactggctgaacggcaaggagtataagtgtaaggtgtccaataaggccctgcctgcccccatcgagaagaccatctccaaggccaagggccagcctcgggagcctcaggtgtataccctgcctccctccagggaggagatgaccaagaatcaggtgtccctgacctgtctggtgaaaggcttctatcccagcgacatcgccgtggagtgggagagcaacggccagcccgagaacaactataagaccaccccccctgtgctggacagcgacggctccttctttctgtacagcaagctgaccgtggataagagcaggtggcagcagggcaacgtgttcagctgcagcgtgatgcacgaggctctgcacaaccactatacccagaagagcctgagcctgtcccctggcaagtga

SEQ ID NO: 76 - DNA, 645 bp, synthetic construct
  misc_feature 1..645: note = anti-C5 (Eculizumab) LC
  source 1..645: mol_type = other DNA
gatatccagatgacccagtccccaagcagcctgagcgccagcgtgggcgaccgggtgaccatcacctgtggcgcttctgagaacatctacggcgccctgaactggtaccagcagaaacccggcaaggcccctaagctgctgatctatggcgctacaaacctggccgacggcgtccccagcagattcagcggcagcggatctggcacagattttaccctgacaattagctccctccaacctgaggacttcgccacctactactgccagaacgtgctgaatacccctctgaccttcggccagggaacaaaggtggaaatcaagaggacagtggccgccccttccgtgttcatctttccaccctctgacgagcagctgaagtctggcaccgccagcgtggtgtgcctgctgaacaacttctacccacgcgaggccaaggtgcagtggaaggtggataacgccctgcagagcggcaattcccaggagtctgtgacagagcaggacagcaaggattccacctattctctgtctagcaccctgacactgagcaaggccgattacgagaagcacaaggtgtatgcctgcgaggtgacacaccagggcctgtcctctcccgtgaccaagtccttcaacaggggcgagtgttga

SEQ ID NO: 77 - DNA, 1989 bp, synthetic construct
  misc_feature 1..1989: note = anti-C3b (MOR09611) HC-hu IgG1 Fc DANG-VEGF binder
  source 1..1989: mol_type = other DNA
gaggtgcagctggtggagagcggcggcggactggtgcagcctggaggatctctgcggctgagctgtgccgctagcggctttaccttcagctcctattggatgacctgggtgaggcaggctcctggcaagggcctggagtgggtgtccagcatcaagatcaagcctgatggctatgctgctagcgtgaagggccggttcaccatctccagggacaacagcaagaacaccctgtacctgcagatgaatagcctgcgggccgaggataccgctgtgtactactgcgccaggctgttctatcagtacttcgctaggatggactattggggccagggcaccctggtgaccgtgagcagcgctagcaccaagggcccctccgtgtttcccctggcccctagctccaagagcaccagcggcggcaccgccgctctgggatgtctggtgaaggactattttcctgagcctgtgaccgtgtcctggaacagcggcgccctgaccagcggcgtgcacacattccccgctgtgctgcagagctccggcctgtactccctgagctccgtggtgaccgtgcctagctccagcctgggcacccagacctacatctgcaatgtgaaccacaagccctccaacaccaaggtggacaagagggtggagcctaagagctgcgacaagacccacacctgccctccttgccccgccccagaggctgctggaggaccttccgtgtttctgttcccccctaagcccaaggataccctgatgatctcccggacccccgaggtgacctgtgtggtggtggctgtgtcccacgaggaccctgaggtgaagtttaactggtacgtggacggcgtggaggtgcacaacgccaagaccaagcccagggaggagcagtacggctccacctacagggtggtgtccgtgctgaccgtgctgcaccaggactggctgaacggcaaggagtataagtgtaaggtgtccaataaggccctgcctgcccccatcgagaagaccatctccaaggccaagggccagcctcgggagcctcaggtgtataccctgcctccctccagggaggagatgaccaagaatcaggtgtccctgacctgtctggtgaaaggcttctatcccagcgacatcgccgtggagtgggagagcaacggccagcccgagaacaactataagaccaccccccctgtgctggacagcgacggctccttctttctgtacagcaagctgaccgtggataagagcaggtggcagcagggcaacgtgttcagctgcagcgtgatgcacgaggctctgcacaaccactatacccagaagagcctgagcctgtcccctggcggaggaggaggcagcggcggtgggggttcctccgatactggcagacccttcgtcgagatgtacagcgagattcctgagatcatccacatgacagagggacgggaactggtgattccttgcagagtgacatctccaaacatcacagtgaccctgaagaagtttcctctggacaccctgatccctgacggcaagcgcatcatctgggacagcagaaagggattcatcatcagcaacgccacctacaaggaaatcggcctcctgacctgcgaggccaccgtgaacggacacctgtataaaaccaattacctgacacaccggcaaacaaacaccatcatcgacgtggtgctgagccctagccacggcatcgagctgagcgtgggcgagaagctggtgctgaactgcaccgccagaaccgaactgaacgtgggcatcgatttcaactgggaatacccctcctctaagcaccagcataagaaactggttaatagagatctgaaaacccagagcggcagcgaaatgaaaaagttcctgtctacactgaccatcgacggcgtgaccagaagcgaccagggcctgtacacctgtgccgcttctagcggcctgatgaccaagaagaacagcacattcgtgcgggtgcacgagaagtga

SEQ ID NO: 78 - DNA, 1986 bp, synthetic construct
  misc_feature 1..1986: note = anti-C3b (MOR09675) HC-hu IgG1 Fc DANG-VEGF binder
  source 1..1986: mol_type = other DNA
gaggtgcagctggtgcagtccggcgccgaggtgaagaagcctggcgctagcgtgaaggtgtcctgcaaggcttccggctacaccttcaccggctactatatcaactgggtgaggcaggctcctggccagggcctggagtggatgggcatcatcagccctaaccagggcaccaccggctacgcccagaagttccagggcagggtgaccatgaccagggacaccagcatcagcaccgcctacatggagctgtccagcctgcggtccgaggacaccgccgtgtactattgtgccaggggcaactacgatcacctggactattggggccagggcaccctggtgaccgtgagctccgctagcaccaagggcccctccgtgtttcccctggcccctagctccaagagcaccagcggcggcaccgccgctctgggatgtctggtgaaggactattttcctgagcctgtgaccgtgtcctggaacagcggcgccctgaccagcggcgtgcacacattccccgctgtgatccagagctccggcctgtactccctgagctccgtggtgaccgtgcctagctccagcctgggcacccagacctacatctgcaatgtgaaccacaagccctccaacaccaaggtggacaagagggtggagcctaagagctgcgacaagacccacacctgccctccttgccccgccccagaggctgctggaggaccttccgtgtttctgttcccccctaagcccaaggataccctgatgatctcccggacccccgaggtgacctgtgtggtggtggctgtgtcccacgaggaccctgaggtgaagtttaactggtacgtggacggcgtggaggtgcacaacgccaagaccaagcccagggaggagcagtacggctccacctacagggtggtgtccgtgctgaccgtgctgcaccaggactggctgaacggcaaggagtataagtgtaaggtgtccaataaggccctgcctgcccccatcgagaagaccatctccaaggccaagggccagcctcgggagcctcaggtgtataccctgcctccctccagggaggagatgaccaagaatcaggtgtccctgacctgtctggtgaaaggcttctatcccagcgacatcgccgtggagtgggagagcaacggccagcccgagaacaactataagaccaccccccctgtgctggacagcgacggctccttctttctgtacagcaagctgaccgtggataagagcaggtggcagcagggcaacgtgttcagctgcagcgtgatgcacgaggctctgcacaaccactatacccagaagagcctgagcctgtcccctggcggaggaggaggcagcggcggtgggggttcctccgatactggcagacccttcgtcgagatgtacagcgagattcctgagatcatccacatgacagagggacgggaactggtgattccttgcagagtgacatctccaaacatcacagtgaccctgaagaagtttcctctggacaccctgatccctgacggcaagcgcatcatctgggacagcagaaagggattcatcatcagcaacgccacctacaaggaaatcggcctcctgacctgcgaggccaccgtgaacggacacctgtataaaaccaattacctgacacaccggcaaacaaacaccatcatcgacgtggtgctgagccctagccacggcatcgagctgagcgtgggcgagaagctggtgctgaactgcaccgccagaaccgaactgaacgtgggcatcgatttcaactgggaatacccctcctctaagcaccagcataagaaactggttaatagagatctgaaaacccagagcggcagcgaaatgaaaaagttcctgtctacactgaccatcgacggcgtgaccagaagcgaccagggcctgtacacctgtgccgcttctagcggcctgatgaccaagaagaacagcacattcgtgcgggtgcacgagaagtga

SEQ ID NO: 79 - DNA, 2004 bp, synthetic construct
  misc_feature 1..2004: note = anti-C3b (S77) HC-hu IgG1 Fc DANG-VEGF binder
  source 1..2004: mol_type = other DNA
gaagtgcagctggttgagagcggcggaggcctcgtgcaacctggcggatctctgcggctgtcttgtgctgcttctggcttcagcttcacctccagcagcgtgtcctgggtgcggcaggcccctggaaaaggcctggaatgggtcggcctgatctacccctacaacggctttaactactacgccgacagcgtgaagggcagattcaccatcagcgccgataccagcaagaacaccgcctacctgcagatgaacagcctgagagccgaggacacagccgtgtactactgcgccagaaatgccctgtacggcagcggcggatattacgccatggactactggggccagggcaccctggtgacagtgtccagcgctagcaccaagggcccctccgtgtttcccctggcccctagctccaagagcaccagcggcggcaccgccgctctgggatgtctggtgaaggactattttcctgagcctgtgaccgtgtcctggaacagcggcgccctgaccagcggcgtgcacacattccccgctgtgatccagagctccggcctgtactccctgagctccgtggtgaccgtgcctagctccagcctgggcacccagacctacatctgcaatgtgaaccacaagccctccaacaccaaggtggacaagagggtggagcctaagagctgcgacaagacccacacctgccctccttgccccgccccagaggctgctggaggaccttccgtgtttctgttcccccctaagcccaaggataccctgatgatctcccggacccccgaggtgacctgtgtggtggtggctgtgtcccacgaggaccctgaggtgaagtttaactggtacgtggacggcgtggaggtgcacaacgccaagaccaagcccagggaggagcagtacggctccacctacagggtggtgtccgtgctgaccgtgctgcaccaggactggctgaacggcaaggagtataagtgtaaggtgtccaataaggccctgcctgcccccatcgagaagaccatctccaaggccaagggccagcctcgggagcctcaggtgtataccctgcctccctccagggaggagatgaccaagaatcaggtgtccctgacctgtctggtgaaaggcttctatcccagcgacatcgccgtggagtgggagagcaacggccagcccgagaacaactataagaccaccccccctgtgctggacagcgacggctccttctttctgtacagcaagctgaccgtggataagagcaggtggcagcagggcaacgtgttcagctgcagcgtgatgcacgaggctctgcacaaccactatacccagaagagcctgagcctgtcccctggcggaggaggaggcagcggcggtgggggttcctccgatactggcagacccttcgtcgagatgtacagcgagattcctgagatcatccacatgacagagggacgggaactggtgattccttgcagagtgacatctccaaacatcacagtgaccctgaagaagtttcctctggacaccctgatccctgacggcaagcgcatcatctgggacagcagaaagggattcatcatcagcaacgccacctacaaggaaatcggcctcctgacctgcgaggccaccgtgaacggacacctgtataaaaccaattacctgacacaccggcaaacaaacaccatcatcgacgtggtgctgagccctagccacggcatcgagctgagcgtgggcgagaagctggtgctgaactgcaccgccagaaccgaactgaacgtgggcatcgatttcaactgggaatacccctcctctaagcaccagcataagaaactggttaatagagatctgaaaacccagagcggcagcgaaatgaaaaagttcctgtctacactgaccatcgacggcgtgaccagaagcgaccagggcctgtacacctgtgccgcttctagcggcctgatgaccaagaagaacagcacattcgtgcgggtgcacgagaagtga

SEQ ID NO: 80 - DNA, 2001 bp, synthetic construct
  misc_feature 1..2001: note = anti-C5 (Eculizumab) HC-hu IgG1 Fc DANG-VEGF binder
  source 1..2001: mol_type = other DNA
caggtgcagctggtgcagagcggcgccgaggtgaagaaacccggagctagcgtgaaggtgtcttgtaaggcctctggctacatcttcagcaattactggatccagtgggtcagacaggcccctggccagggcctggaatggatgggcgagatcctgcctggaagcggctctaccgagtacaccgaaaacttcaaggacagagtgaccatgacccgggataccagcacaagcaccgtttacatggaactgagctccctgcggagcgaggacacagccgtgtattactgcgccagatactttttcggcagctccccaaactggtacttcgacgtgtggggccaaggcaccctggtgacagtgtccagcgctagcaccaagggcccctccgtgtttcccctggcccctagctccaagagcaccagcggcggcaccgccgctctgggatgtctggtgaaggactattttcctgagcctgtgaccgtgtcctggaacagcggcgccctgaccagcggcgtgcacacattccccgctgtgatccagagctccggcctgtactccctgagctccgtggtgaccgtgcctagctccagcctgggcacccagacctacatctgcaatgtgaaccacaagccctccaacaccaaggtggacaagagggtggagcctaagagctgcgacaagacccacacctgccctccttgccccgccccagaggctgctggaggaccttccgtgtttctgttcccccctaagcccaaggataccctgatgatctcccggacccccgaggtgacctgtgtggtggtggctgtgtcccacgaggaccctgaggtgaagtttaactggtacgtggacggcgtggaggtgcacaacgccaagaccaagcccagggaggagcagtacggctccacctacagggtggtgtccgtgctgaccgtgctgcaccaggactggctgaacggcaaggagtataagtgtaaggtgtccaataaggccctgcctgcccccatcgagaagaccatctccaaggccaagggccagcctcgggagcctcaggtgtataccctgcctccctccagggaggagatgaccaagaatcaggtgtccctgacctgtctggtgaaaggcttctatcccagcgacatcgccgtggagtgggagagcaacggccagcccgagaacaactataagaccaccccccctgtgctggacagcgacggctccttctttctgtacagcaagctgaccgtggataagagcaggtggcagcagggcaacgtgttcagctgcagcgtgatgcacgaggctctgcacaaccactatacccagaagagcctgagcctgtcccctggcggaggaggaggcagcggcggtgggggttcctccgatactggcagacccttcgtcgagatgtacagcgagattcctgagatcatccacatgacagagggacgggaactggtgattccttgcagagtgacatctccaaacatcacagtgaccctgaagaagtttcctctggacaccctgatccctgacggcaagcgcatcatctgggacagcagaaagggattcatcatcagcaacgccacctacaaggaaatcggcctcctgacctgcgaggccaccgtgaacggacacctgtataaaaccaattacctgacacaccggcaaacaaacaccatcatcgacgtggtgctgagccctagccacggcatcgagctgagcgtgggcgagaagctggtgctgaactgcaccgccagaaccgaactgaacgtgggcatcgatttcaactgggaatacccctcctctaagcaccagcataagaaactggttaatagagatctgaaaacccagagcggcagcgaaatgaaaaagttcctgtctacactgaccatcgacggcgtgaccagaagcgaccagggcctgtacacctgtgccgcttctagcggcctgatgaccaagaagaacagcacattcgtgcgggtgcacgagaagtga

SEQ ID NO: 81 - DNA, 2091 bp, synthetic construct
  misc_feature 1..2091: note = VEGF binder-hu IgG1 Fc DANG-anti-C3b (MOR09611) scFv
  source 1..2091: mol_type = other DNA
tccgatactggcagacccttcgtcgagatgtacagcgagattcctgagatcatccacatgacagagggacgggaactggtgattccttgcagagtgacatctccaaacatcacagtgaccctgaagaagtttcctctggacaccctgatccctgacggcaagcgcatcatctgggacagcagaaagggattcatcatcagcaacgccacctacaaggaaatcggcctcctgacctgcgaggccaccgtgaacggacacctgtataaaaccaattacctgacacaccggcaaacaaacaccatcatcgacgtggtgctgagccctagccacggcatcgagctgagcgtgggcgagaagctggtgctgaactgcaccgccagaaccgaactgaacgtgggcatcgatttcaactgggaatacccctcctctaagcaccagcataagaaactggttaatagagatctgaaaacccagagcggcagcgaaatgaaaaagttcctgtctacactgaccatcgacggcgtgaccagaagcgaccagggcctgtacacctgtgccgcttctagcggcctgatgaccaagaagaacagcacattcgtgcgggtgcacgagaagggaggaggcggcagcgataagacccacacatgcccaccctgtcctgcaccagaggcagccggaggaccatccgtgttcctgtttcctccaaagcctaaggacaccctgatgatctctcggaccccagaggtgacatgcgtggtggtggccgtgagccacgaggaccccgaggtgaagtttaactggtacgtggatggcgtggaggtgcacaatgccaagaccaagccccgggaggagcagtacggctccacctatagagtggtgtctgtgctgacagtgctgcaccaggattggctgaacggcaaggagtataagtgcaaggtgtccaataaggccctgcccgcccctatcgagaagaccatctctaaggcaaagggacagccaagggagccacaggtgtacacactgcccccttccagagaggagatgaccaagaaccaggtgtctctgacatgtctggtgaagggcttctatccctctgatatcgccgtggagtgggagagcaatggccagcctgagaacaattacaagaccacaccacccgtgctggactccgatggctctttctttctgtatagcaagctgaccgtggataagtccagatggcagcagggcaacgtgttttcttgtagcgtgatgcacgaggccctgcacaatcactacacacagaagtccctgtctctgagccccggcggaggtggaggctcaggtggtggcggatctggaggaggcggtagtgaggtgcagctggtggagagcggcggcggactggtgcagcctggaggatctctgcggctgagctgtgccgctagcggctttaccttcagctcctattggatgacctgggtgaggcaggctcctggcaagggcctggagtgggtgtccagcatcaagatcaagcctgatggctatgctgctagcgtgaagggccggttcaccatctccagggacaacagcaagaacaccctgtacctgcagatgaatagcctgcgggccgaggataccgctgtgtactactgcgccaggctgttctatcagtacttcgctaggatggactattggggccagggcaccctggtgaccgtgagcagcggcggcgggggcagcggtggtggcggatctgggggaggaggtagcggtgggggcggttctgacatccagatgacccagagccccagcagcctgagcgccagcgtgggagatcgggtgaccatcacctgtagggccagccaggatatcagcaattatctgaattggtaccagcagaagcccggcaaggctcccaagctgctgatctacgccgcttccaatctgcagtccggcgtgcccagcaggttcagcggctccggaagcggcaccgactttaccctgaccatctccagcctgcagcccgaggattttgctacctactactgccagcagcacgacaccttcaggcctaccttcggccagggcaccaaggtggagatcaagtga

SEQ ID NO: 82 - DNA, 2091 bp, synthetic construct
  misc_feature 1..2091: note = VEGF binder-hu IgG1 Fc DANG-anti-C3b (MOR09675) scFv
  source 1..2091: mol_type = other DNA
tccgatactggcagacccttcgtcgagatgtacagcgagattcctgagatcatccacatgacagagggacgggaactggtgattccttgcagagtgacatctccaaacatcacagtgaccctgaagaagtttcctctggacaccctgatccctgacggcaagcgcatcatctgggacagcagaaagggattcatcatcagcaacgccacctacaaggaaatcggcctcctgacctgcgaggccaccgtgaacggacacctgtataaaaccaattacctgacacaccggcaaacaaacaccatcatcgacgtggtgctgagccctagccacggcatcgagctgagcgtgggcgagaagctggtgctgaactgcaccgccagaaccgaactgaacgtgggcatcgatttcaactgggaatacccctcctctaagcaccagcataagaaactggttaatagagatctgaaaacccagagcggcagcgaaatgaaaaagttcctgtctacactgaccatcgacggcgtgaccagaagcgaccagggcctgtacacctgtgccgcttctagcggcctgatgaccaagaagaacagcacattcgtgcgggtgcacgagaagggaggaggcggcagcgataagacccacacatgcccaccctgtcctgcaccagaggcagccggaggaccatccgtgttcctgtttcctccaaagcctaaggacaccctgatgatctctcggaccccagaggtgacatgcgtggtggtggccgtgagccacgaggaccccgaggtgaagtttaactggtacgtggatggcgtggaggtgcacaatgccaagaccaagccccgggaggagcagtacggctccacctatagagtggtgtctgtgctgacagtgctgcaccaggattggctgaacggcaaggagtataagtgcaaggtgtccaataaggccctgcccgcccctatcgagaagaccatctctaaggcaaagggacagccaagggagccacaggtgtacacactgcccccttccagagaggagatgaccaagaaccaggtgtctctgacatgtctggtgaagggcttctatccctctgatatcgccgtggagtgggagagcaatggccagcctgagaacaattacaagaccacaccacccgtgctggactccgatggctctttctttctgtatagcaagctgaccgtggataagtccagatggcagcagggcaacgtgttttcttgtagcgtgatgcacgaggccctgcacaatcactacacacagaagtccctgtctctgagccccggcggaggtggaggctcaggtggtggcggatctggaggaggcggtagtgaggtgcagctggtgcagtccggcgccgaggtgaagaagcctggcgctagcgtgaaggtgtcctgcaaggcttccggctacaccttcaccggctactatatcaactgggtgaggcaggctcctggccagggcctggagtggatgggcatcatcagccctaaccagggcaccaccggctacgcccagaagttccagggcagggtgaccatgaccagggacaccagcatcagcaccgcctacatggagctgtccagcctgcggtccgaggacaccgccgtgtactattgtgccaggggcaactacgatcacctggactattggggccagggcaccctggtgaccgtgagctccggcggcgggggcagcggtggtggcggatctgggggaggaggtagcggtgggggcggttctgatatccagatgacccagtcccccagcagcctgagcgcctccgtgggagatcgggtgaccatcacctgtagggcctcccagggcatcagcaactatctgaattggtaccagcagaagcccggcaaggctcccaagctgctgatctacgacgctagcaccctgcagtccggcgtgccctccagattcagcggcagcggctccggcaccgacttcaccctgaccatcagctccctgcagcctgaggatttcgccacctactattgtcagcaggactggcacaccctgcctgtgaccttcggccagggcaccaaggtggagatcaagtga

SEQ ID NO: 83 - DNA, 2106 bp, synthetic construct
  misc_feature 1..2106: note = VEGF binder-hu IgG1 Fc DANG-anti-C3b (S77) scFv
  source 1..2106: mol_type = other DNA
tccgatactggcagacccttcgtcgagatgtacagcgagattcctgagatcatccacatgacagagggacgggaactggtgattccttgcagagtgacatctccaaacatcacagtgaccctgaagaagtttcctctggacaccctgatccctgacggcaagcgcatcatctgggacagcagaaagggattcatcatcagcaacgccacctacaaggaaatcggcctcctgacctgcgaggccaccgtgaacggacacctgtataaaaccaattacctgacacaccggcaaacaaacaccatcatcgacgtggtgctgagccctagccacggcatcgagctgagcgtgggcgagaagctggtgctgaactgcaccgccagaaccgaactgaacgtgggcatcgatttcaactgggaatacccctcctctaagcaccagcataagaaactggttaatagagatctgaaaacccagagcggcagcgaaatgaaaaagttcctgtctacactgaccatcgacggcgtgaccagaagcgaccagggcctgtacacctgtgccgcttctagcggcctgatgaccaagaagaacagcacattcgtgcgggtgcacgagaagggaggaggcggcagcgataagacccacacatgcccaccctgtcctgcaccagaggcagccggaggaccatccgtgttcctgtttcctccaaagcctaaggacaccctgatgatctctcggaccccagaggtgacatgcgtggtggtggccgtgagccacgaggaccccgaggtgaagtttaactggtacgtggatggcgtggaggtgcacaatgccaagaccaagccccgggaggagcagtacggctccacctatagagtggtgtctgtgctgacagtgctgcaccaggattggctgaacggcaaggagtataagtgcaaggtgtccaataaggccctgcccgcccctatcgagaagaccatctctaaggcaaagggacagccaagggagccacaggtgtacacactgcccccttccagagaggagatgaccaagaaccaggtgtctctgacatgtctggtgaagggcttctatccctctgatatcgccgtggagtgggagagcaatggccagcctgagaacaattacaagaccacaccacccgtgctggactccgatggctctttctttctgtatagcaagctgaccgtggataagtccagatggcagcagggcaacgtgttttcttgtagcgtgatgcacgaggccctgcacaatcactacacacagaagtccctgtctctgagccccggcggaggtggaggctcaggtggtggcggatctggaggaggcggtagtgaagtgcagctggttgagagcggcggaggcctcgtgcaacctggcggatctctgcggctgtcttgtgctgcttctggcttcagcttcacctccagcagcgtgtcctgggtgcggcaggcccctggaaaaggcctggaatgggtcggcctgatctacccctacaacggctttaactactacgccgacagcgtgaagggcagattcaccatcagcgccgataccagcaagaacaccgcctacctgcagatgaacagcctgagagccgaggacacagccgtgtactactgcgccagaaatgccctgtacggcagcggcggatattacgccatggactactggggccagggcaccctggtgacagtgtccagcggcggcgggggcagcggtggtggcggatctgggggaggaggtagcggtgggggcggttctgatatccagatgacacagagcccaagcagcctgagcgcttctgtgggcgaccgggtgaccatcacatgtagagccagccaggacgtgtccaccgccgtggcctggtaccagcagaaacccggcaaggcccctaagctgctgatctactccgctagcttcctgtacagcggcgtccccagcagattcagcggatctggcagcggcacagattttaccctgaccatcagctccctgcagcctgaggacttcgccacctactactgccagcaatcttatgccacactgcctaccttcgagcagggcaccaaggtggaaatcaagtga

SEQ ID NO: 84 - DNA, 2100 bp, synthetic construct
  misc_feature 1..2100: note = VEGF binder-hu IgG1 Fc DANG-anti-C5 (Eculizumab) scFv
  source 1..2100: mol_type = other DNA
tccgatactggcagacccttcgtcgagatgtacagcgagattcctgagatcatccacatgacagagggacgggaactggtgattccttgcagagtgacatctccaaacatcacagtgaccctgaagaagtttcctctggacaccctgatccctgacggcaagcgcatcatctgggacagcagaaagggattcatcatcagcaacgccacctacaaggaaatcggcctcctgacctgcgaggccaccgtgaacggacacctgtataaaaccaattacctgacacaccggcaaacaaacaccatcatcgacgtggtgctgagccctagccacggcatcgagctgagcgtgggcgagaagctggtgctgaactgcaccgccagaaccgaactgaacgtgggcatcgatttcaactgggaatacccctcctctaagcaccagcataagaaactggttaatagagatctgaaaacccagagcggcagcgaaatgaaaaagttcctgtctacactgaccatcgacggcgtgaccagaagcgaccagggcctgtacacctgtgccgcttctagcggcctgatgaccaagaagaacagcacattcgtgcgggtgcacgagaagggaggaggcggcagcgataagacccacacatgcccaccctgtcctgcaccagaggcagccggaggaccatccgtgttcctgtttcctccaaagcctaaggacaccctgatgatctctcggaccccagaggtgacatgcgtggtggtggccgtgagccacgaggaccccgaggtgaagtttaactggtacgtggatggcgtggaggtgcacaatgccaagaccaagccccgggaggagcagtacggctccacctatagagtggtgtctgtgctgacagtgctgcaccaggattggctgaacggcaaggagtataagtgcaaggtgtccaataaggccctgcccgcccctatcgagaagaccatctctaaggcaaagggacagccaagggagccacaggtgtacacactgcccccttccagagaggagatgaccaagaaccaggtgtctctgacatgtctggtgaagggcttctatccctctgatatcgccgtggagtgggagagcaatggccagcctgagaacaattacaagaccacaccacccgtgctggactccgatggctctttctttctgtatagcaagctgaccgtggataagtccagatggcagcagggcaacgtgttttcttgtagcgtgatgcacgaggccctgcacaatcactacacacagaagtccctgtctctgagccccggcggaggtggaggctcaggtggtggcggatctggaggaggcggtagtatggccgatatccagatgacccagtccccaagcagcctgagcgccagcgtgggcgaccgggtgaccatcacctgtggcgcttctgagaacatctacggcgccctgaactggtaccagcagaaacccggcaaggcccctaagctgctgatctatggcgctacaaacctggccgacggcgtccccagcagattcagcggcagcggatctggcacagattttaccctgacaattagctccctccaacctgaggacttcgccacctactactgccagaacgtgctgaatacccctctgaccttcggccagggaacaaaggtggaaatcaagaggacaggcggcgggggcagcggtggtggcggatctgggggaggaggtagccaggtgcagctggtgcagagcggcgccgaggtgaagaaacccggagctagcgtgaaggtgtcttgtaaggcctctggctacatcttcagcaattactggatccagtgggtcagacaggcccctggccagggcctggaatggatgggcgagatcctgcctggaagcggctctaccgagtacaccgaaaacttcaaggacagagtgaccatgacccgggataccagcacaagcaccgtttacatggaactgagctccctgcggagcgaggacacagccgtgtattactgcgccagatactttttcggcagctccccaaactggtacttcgacgtgtggggccaaggcaccctggtgacagtgtccagctga

SEQ ID NO: 85 - DNA, 678 bp, synthetic construct
  misc_feature 1..678: note = hu IgG1 Fc DANG
  source 1..678: mol_type = other DNA
gacaagacccacacatgcccaccttgtccagcaccagagctgctgggaggaccatccgtgttcctgtttccacccaagcccaaggataccctgatgatcagcaggaccccagaggtgacatgcgtggtggtggccgtgtcccacgaggaccctgaggtgaagttcaactggtacgtggatggcgtggaggtgcacaatgccaagaccaagccacgggaggagcagtacggctccacctatagagtggtgtctgtgctgacagtgctgcaccaggactggctgaacggcaaggagtataagtgcaaggtgtctaataaggccctgcctgccccaatcgagaagaccatcagcaaggcaaagggacagccaagggagcctcaggtgtacacactgcctccatcccgcgacgagctgaccaagaaccaggtgtctctgacatgtctggtgaagggcttctatccttctgatatcgccgtggagtgggagagcaatggccagccagagaacaattacaagaccacaccccctgtgctggactctgatggcagcttctttctgtatagcaagctgaccgtggataagtccaggtggcagcagggcaacgtgtttagctgttccgtgatgcacgaggccctgcacaatcactacacacagaagtctctgagcctgtcccctggc

SEQ ID NO: 86 - DNA, 2130 bp, synthetic construct
  misc_feature 1..2130: note = hu CRIg-hu IgG1 Fc DANG-VEGF binder
  source 1..2130: mol_type = other DNA
cgccctatcctggaggtgccagagtccgtgaccggaccatggaagggcgacgtgaacctgccctgcacctacgatcctctgcagggctatacacaggtgctggtgaagtggctggtgcagaggggcagcgaccctgtgaccatcttcctgcgcgacagctccggcgatcacatccagcaggccaagtaccagggcaggctgcacgtgtcccacaaggtgcctggcgacgtgagcctgcagctgtctaccctggagatggacgatcgcagccactatacatgtgaggtgacctggcagacaccagacggcaatcaggtggtgagggataagatcaccgagctgcgcgtgcagaagctgtccgtgtctaagccaaccgtgaccacaggctctggctacggcttcacagtgccccagggcatgaggatcagcctgcagtgccaggcaaggggcagcccacctatctcctacatctggtataagcagcagaccaacaatcaggagcctatcaaggtggccaccctgtccacactgctgttcaagccagccgtgatcgccgacagcggctcctacttttgtacagccaagggccaagtgggctctgagcagcacagcgacatcgtgaagtttgtggtgaaggattctagcaagctgctgaagaccaagacagaggcccctaccacaatgacctacccactgaaggccacctccacagtgaagcagtcttgggactggaccacagacatggatggctatctgggagagacaagcgccggacctggcaagtccctgccaggaggcggcggctccgataagacccacacatgcccaccatgtcctgcaccagagctgctgggaggacctagcgtgttcctgtttcctccaaagccaaaggacaccctgatgatctcccggaccccagaggtgacatgcgtggtggtggccgtgtctcacgaggaccccgaggtgaagttcaactggtacgtggatggcgtggaggtgcacaatgccaagaccaagccccgggaggagcagtacggctctacctatagagtggtgagcgtgctgacagtgctgcaccaggattggctgaacggcaaggagtataagtgcaaggtgagcaataaggccctgcccgcccctatcgagaagaccatctccaaggcaaagggacagccaagggagccacaggtgtacacactgcccccttccagagacgagctgaccaagaaccaggtgtctctgacatgtctggtgaagggcttttatccctctgatatcgccgtggagtgggagagcaatggccagcctgagaacaattacaagaccacaccacccgtgctggactctgatggcagcttctttctgtattccaagctgaccgtggacaagtctagatggcagcagggcaacgtgttctcttgcagcgtgatgcacgaggccctgcacaatcactacacccagaagtccctgtctctgagcccaggaggaggaggaggctctggaggaggaggctcctctgatacaggcaggccctttgtggagatgtatagcgagatccctgagatcatccacatgaccgagggaagggagctggtcatcccatgtagagtgacatcccctaacatcaccgtgacactgaagaagttcccactggacaccctgatccccgatggcaagcggatcatctgggacagcagaaagggctttatcatctccaatgccacatacaaggagatcggcctgctgacctgcgaggccacagtgaacggccacctgtacaagaccaattatctgacacaccgccagaccaacacaatcatcgatgtggtgctgtccccatctcacggcatcgagctgagcgtgggcgagaagctggtgctgaattgtaccgcccggacagagctgaacgtgggcatcgacttcaattgggagtaccctagctccaagcaccagcacaagaagctggtcaaccgggatctgaagacccagagcggctccgagatgaagaagtttctgagcaccctgacaatcgacggcgtgaccagatccgatcagggcctgtatacatgtgccgcctctagcggcctgatgaccaagaagaatagcacatttgtgagggtgcacgagaag

SEQ ID NO: 87 - DNA, 1293 bp, synthetic construct
  misc_feature 1..1293: note = VEGF binder-hu IgG1 Fc
  source 1..1293: mol_type = other DNA
tccgatactggcagacccttcgtcgagatgtacagcgagattcctgagatcatccacatgacagagggacgggaactggtgattccttgcagagtgacatctccaaacatcacagtgaccctgaagaagtttcctctggacaccctgatccctgacggcaagcgcatcatctgggacagcagaaagggattcatcatcagcaacgccacctacaaggaaatcggcctcctgacctgcgaggccaccgtgaacggacacctgtataaaaccaattacctgacacaccggcaaacaaacaccatcatcgacgtggtgctgagccctagccacggcatcgagctgagcgtgggcgagaagctggtgctgaactgcaccgccagaaccgaactgaacgtgggcatcgatttcaactgggaatacccctcctctaagcaccagcataagaaactggttaatagagatctgaaaacccagagcggcagcgaaatgaaaaagttcctgtctacactgaccatcgacggcgtgaccagaagcgaccagggcctgtacacctgtgccgcttctagcggcctgatgaccaagaagaacagcacattcgtgcgggtgcacgagaaggacaaaactcacacatgcccaccgtgcccagcacctgaactcctggggggaccgtcagtcttcctcttccccccaaaacccaaggacaccctcatgatctcccggacccctgaggtcacatgcgtggtggtggacgtgagccacgaagaccctgaggtcaagttcaactggtacgtggacggcgtggaggtgcataatgccaagacaaagccgcgggaggagcagtacaacagcacgtaccgtgtggtcagcgtcctcaccgtcctgcaccaggactggctgaatggcaaggagtacaagtgcaaggtctccaacaaagccctcccagcccccatcgagaaaaccatctccaaagccaaagggcagccccgagaaccacaggtgtacaccctgcccccatcccgggatgagctgaccaagaaccaggtcagcctgacctgcctggtcaaaggcttctatcccagcgacatcgccgtggagtgggagagcaatgggcagccggagaacaactacaagaccacgcctcccgtgctggactccgacggctccttcttcctctacagcaagctcaccgtggacaagagcaggtggcagcaggggaacgtcttctcatgctccgtgatgcatgaggctctgcacaaccactacacgcagaagagcctctccctgtctccgggt

SEQ ID NO: 88 - protein, 5 aa, synthetic construct
  REGION 1..5: note = CDR1 of anti-VEGF VHH-antibody BI-836880
SYSMG

SEQ ID NO: 89 - protein, 16 aa, synthetic construct
  REGION 1..16: note = CDR2 of anti-VEGF VHH-antibody BI-836880
AISKGGYKYDAVSLEG

SEQ ID NO: 90 - protein, 17 aa, synthetic construct
  REGION 1..17: note = CDR3 of anti-VEGF VHH-antibody BI-836880
SRAYGSSRLRLADTYEY

SEQ ID NO: 91 - protein, 10 aa, synthetic construct
  REGION 1..10: note = HCDR1 of Bevacizumab
GYTFTNYGMN

SEQ ID NO: 92 - protein, 17 aa, synthetic construct
  REGION 1..17: note = HCDR2 of Bevacizumab
WINTYTGEPTYAADFKR

SEQ ID NO: 93 - protein, 14 aa, synthetic construct
  REGION 1..14: note = HCDR3 of Bevacizumab
YPHYYGSSHWYFDV

SEQ ID NO: 94 - protein, 11 aa, synthetic construct
  REGION 1..11: note = LCDR1 of Bevacizumab
SASQDISNYLN

SEQ ID NO: 95 - protein, 7 aa, synthetic construct
  REGION 1..7: note = LCDR2 of Bevacizumab
FTSSLHS

SEQ ID NO: 96 - protein, 9 aa, synthetic construct
  REGION 1..9: note = LCDR3 of Bevacizumab
QQYSTVPWT

SEQ ID NO: 97 - protein, 10 aa, synthetic construct
  REGION 1..10: note = HCDR1 of Ranibizumab
GYDFTHYGMN

SEQ ID NO: 98 - protein, 17 aa, synthetic construct
  REGION 1..17: note = HCDR2 of Ranibizumab
WINTYTGEPTYAADFKR

SEQ ID NO: 99 - protein, 14 aa, synthetic construct
  REGION 1..14: note = HCDR3 of Ranibizumab
YPYYYGTSHWYFDV

SEQ ID NO: 100 - protein, 11 aa, synthetic construct
  REGION 1..11: note = LCDR1 of Ranibizumab
SASQDISNYLN

SEQ ID NO: 101 - protein, 7 aa, synthetic construct
  REGION 1..7: note = LCDR2 of Ranibizumab
FTSSLHS

SEQ ID NO: 102 - protein, 9 aa, synthetic construct
  REGION 1..9: note = LCDR3 of Ranibizumab
QQYSTVPWT

SEQ ID NO: 103 - protein, 10 aa, synthetic construct
  REGION 1..10: note = HCDR1 of Ramucirumab
GFTFSSYSMN

SEQ ID NO: 104 - protein, 17 aa, synthetic construct
  REGION 1..17: note = HCDR2 of Ramucirumab
SISSSSSYIYYADSVKG

SEQ ID NO: 105 - protein, 7 aa, synthetic construct
  REGION 1..7: note = HCDR3 of Ramucirumab
VTDAFDI

SEQ ID NO: 106 - protein, 11 aa, synthetic construct
  REGION 1..11: note = LCDR1 of Ramucirumab
RASQGIDNWLG

SEQ ID NO: 107 - protein, 7 aa, synthetic construct
  REGION 1..7: note = LCDR2 of Ramucirumab
DASNLDT

SEQ ID NO: 108 - protein, 9 aa, synthetic construct
  REGION 1..9: note = LCDR3 of Ramucirumab
QQAKAFPPT

SEQ ID NO: 109 - protein, 10 aa, synthetic construct
  REGION 1..10: note = HCDR1 of Faricimab
GYDFTHYGMN

SEQ ID NO: 110 - protein, 17 aa, synthetic construct
  REGION 1..17: note = HCDR2 of Faricimab
WINTYTGEPTYAADFKR

SEQ ID NO: 111 - protein, 14 aa, synthetic construct
  REGION 1..14: note = HCDR3 of Faricimab
YPYYYGTSHWYFDV

SEQ ID NO: 112 - protein, 11 aa, synthetic construct
  REGION 1..11: note = LCDR1 of Faricimab
SASQDISNYLN

SEQ ID NO: 113 - protein, 7 aa, synthetic construct
  REGION 1..7: note = LCDR2 of Faricimab
FTSSLHS

SEQ ID NO: 114 - protein, 9 aa, synthetic construct
  REGION 1..9: note = LCDR3 of Faricimab
QQYSTVPWT

SEQ ID NO: 115 - protein, 10 aa, synthetic construct
  REGION 1..10: note = HCDR1 of KSI-301
GYDFTHYGMN

SEQ ID NO: 116 - protein, 17 aa, synthetic construct
  REGION 1..17: note = HCDR2 of KSI-301
WINTYTGEPTYAADFKR

SEQ ID NO: 117 - protein, 14 aa, synthetic construct
  REGION 1..14: note = HCDR3 of KSI-301
YPYYYGTSHWYFDV

SEQ ID NO: 118 - protein, 11 aa, synthetic construct
  REGION 1..11: note = LCDR1 of KSI-301
SASQDISNYLN

SEQ ID NO: 119 - protein, 7 aa, synthetic construct
  REGION 1..7: note = LCDR2 of KSI-301
FTSSLHS

SEQ ID NO: 120 - protein, 9 aa, synthetic construct
  REGION 1..9: note = LCDR3 of KSI-301
QQYSTVPWT

SEQ ID NO: 121 - protein, 10 aa, synthetic construct
  REGION 1..10: note = HCDR1 of Vanucizumab
GYTFTNYGMN

SEQ ID NO: 122 - protein, 17 aa, synthetic construct
  REGION 1..17: note = HCDR2 of Vanucizumab
WINTYTGEPTYAADFKR

SEQ ID NO: 123 - protein, 14 aa, synthetic construct
  REGION 1..14: note = HCDR3 of Vanucizumab
YPHYYGSSHWYFDV

SEQ ID NO: 124 - protein, 11 aa, synthetic construct
  REGION 1..11: note = LCDR1 of Vanucizumab
SASQDISNYLN

SEQ ID NO: 125 - protein, 7 aa, synthetic construct
  REGION 1..7: note = LCDR2 of Vanucizumab
FTSSLHS

SEQ ID NO: 126 - protein, 9 aa, synthetic construct
  REGION 1..9: note = LCDR3 of Vanucizumab
QQYSTVPWT

SEQ ID NO: 127 - protein, 10 aa, synthetic construct
  REGION 1..10: note = HCDR1 of BAT-5906
GYDFTHYGMN

SEQ ID NO: 128 - protein, 17 aa, synthetic construct
  REGION 1..17: note = HCDR2 of BAT-5906
WINTYTGEPTYAADFKR

SEQ ID NO: 129 - protein, 14 aa, synthetic construct
  REGION 1..14: note = HCDR3 of BAT-5906
YPYYYGTSHWYFDV

SEQ ID NO: 130 - protein, 11 aa, synthetic construct
  REGION 1..11: note = LCDR1 of BAT-5906
SASQDISNYLN

SEQ ID NO: 131 - protein, 7 aa, synthetic construct
  REGION 1..7: note = LCDR2 of BAT-5906
FTSSLHS

SEQ ID NO: 132 - protein, 10 aa, synthetic construct
  REGION 1..10: note = LCDR3 of BAT-5906
CQQYSTVPWT

SEQ ID NO: 133 - protein, 5 aa, synthetic construct
  REGION 1..5: note = HCDR1 of Navicixizumab
NYWMH

SEQ ID NO: 134 - protein, 17 aa, synthetic construct
  REGION 1..17: note = HCDR2 of Navicixizumab
DINPSNGRTSYKEKFKR

SEQ ID NO: 135 - protein, 12 aa, synthetic construct
  REGION 1..12: note = HCDR3 of Navicixizumab
HYDDKYYPLMDY

SEQ ID NO: 136 - protein, 15 aa, synthetic construct
  REGION 1..15: note = LCDR1 of Navicixizumab
RASESVDNYGISFMK

SEQ ID NO: 137 - protein, 7 aa, synthetic construct
  REGION 1..7: note = LCDR2 of Navicixizumab
AASNQGS

SEQ ID NO: 138 - protein, 12 aa, synthetic construct
  REGION 1..12: note = LCDR3 of Navicixizumab
QQSKEVPWTFGG

SEQ ID NO: 139 - protein, 11 aa, synthetic construct
  REGION 1..11: note = HCDR1 of Dilpacimab
SGYTFTNYGMN

SEQ ID NO: 140 - protein, 16 aa, synthetic construct
  REGION 1..16: note = HCDR2 of Dilpacimab
INTYTGEPTYAADFKR

SEQ ID NO: 141 - protein, 14 aa, synthetic construct
  REGION 1..14: note = HCDR3 of Dilpacimab
YPHYYGSSHWYFDV

SEQ ID NO: 142 - protein, 11 aa, synthetic construct
  REGION 1..11: note = LCDR1 of Dilpacimab
SASQDISNYLN

SEQ ID NO: 143 - protein, 7 aa, synthetic construct
  REGION 1..7: note = LCDR2 of Dilpacimab
FTSSLHS

SEQ ID NO: 144 - protein, 8 aa, synthetic construct
  REGION 1..8: note = LCDR3 of Dilpacimab
QQYSTVPW

SEQ ID NO: 145 - protein, 10 aa, synthetic construct
  REGION 1..10: note = HCDR1 of hPV-19
GYSFTNSGIN

SEQ ID NO: 146 - protein, 14 aa, synthetic construct
  REGION 1..14: note = HCDR2 of hPV-19
INTYTGEPTYADDF

SEQ ID NO: 147 - protein, 10 aa, synthetic construct
  REGION 1..10: note = HCDR3 of hPV-19
FGDGYYWFFD

SEQ ID NO: 148 - protein, 17 aa, synthetic construct
  REGION 1..17: note = LCDR1 of hPV-19
KSSQSLLNSRTRKNFLA

SEQ ID NO: 149 - protein, 7 aa, synthetic construct
  REGION 1..7: note = LCDR2 of hPV-19
WASTRES

SEQ ID NO: 150 - protein, 11 aa, synthetic construct
  REGION 1..11: note = LCDR3 of hPV-19
KQSYNLYTFGG

SEQ ID NO: 151 - protein, 5 aa, synthetic construct
  REGION 1..5: note = HCDR1 of AT-001
SYAIS

SEQ ID NO: 152 - protein, 17 aa, synthetic construct
  REGION 1..17: note = HCDR2 of AT-001
GFDPEDGETIYAQKFQG

SEQ ID NO: 153 - protein, 17 aa, synthetic construct
  REGION 1..17: note = HCDR3 of AT-001
GRSMVRGVIIPFNGMDV

SEQ ID NO: 154 - protein, 11 aa, synthetic construct
  REGION 1..11: note = LCDR1 of AT-001
RASQSISSYLN

SEQ ID NO: 155 - protein, 7 aa, synthetic construct
  REGION 1..7: note = LCDR2 of AT-001
AASSLQS

SEQ ID NO: 156 - protein, 9 aa, synthetic construct
  REGION 1..9: note = LCDR3 of AT-001
QQSYSTPLT

SEQ ID NO: 157 - protein, 453 aa, synthetic construct
  REGION 1..453: note = Heavy chain of anti-VEGF antibody Bevacizumab
EVQLVESGGGLVQPGGSLRLSCAASGYTFTNYGMNWVRQAPGKGLEWVGWINTYTGEPTYAADFKRRFTFSLDTSKSTAYLQMNSLRAEDTAVYYCAKYPHYYGSSHWYFDVWGQGTLVTVSSASTKGPSVFPLAPSSKSTSGGTAALGCLVKDYFPEPVTVSWNSGALTSGVHTFPAVLQSSGLYSLSSVVTVPSSSLGTQTYICNVNHKPSNTKVDKKVEPKSCDKTHTCPPCPAPELLGGPSVFLFPPKPKDTLMISRTPEVTCVVVDVSHEDPEVKFNWYVDGVEVHNAKTKPREEQYNSTYRVVSVLTVLHQDWLNGKEYKCKVSNKALPAPIEKTISKAKGQPREPQVYTLPPSREEMTKNQVSLTCLVKGFYPSDIAVEWESNGQPENNYKTTPPVLDSDGSFFLYSKLTVDKSRWQQGNVFSCSVMHEALHNHYTQKSLSLSPGK

SEQ ID NO: 158 - protein, 214 aa, synthetic construct
  REGION 1..214: note = Light chain of anti-VEGF antibody Bevacizumab
DIQMTQSPSSLSASVGDRVTITCSASQDISNYLNWYQQKPGKAPKVLIYFTSSLHSGVPSRFSGSGSGTDFTLTISSLQPEDFATYYCQQYSTVPWTFGQGTKVEIKRTVAAPSVFIFPPSDEQLKSGTASVVCLLNNFYPREAKVQWKVDNALQSGNSQESVTEQDSKDSTYSLSSTLTLSKADYEKHKVYACEVTHQGLSSPVTKSFNRGEC

SEQ ID NO: 159 - protein, 231 aa, synthetic construct
  REGION 1..231: note = Variable Heavy chain of anti-VEGF antibody Ranibizumab
EVQLVESGGGLVQPGGSLRLSCAASGYDFTHYGMNWVRQAPGKGLEWVGWINTYTGEPTYAADFKRRFTFSLDTSKSTAYLQMNSLRAEDTAVYYCAKYPYYYGTSHWYFDVWGQGTLVTVSSASTKGPSVFPLAPSSKSTSGGTAALGCLVKDYFPEPVTVSWNSGALTSGVHTFPAVLQSSGLYSLSSVVTVPSSSLGTQTYICNVNHKPSNTKVDKKVEPKSCDKTHL

SEQ ID NO: 160 - protein, 214 aa, synthetic construct
  REGION 1..214: note = Light chain of anti-VEGF antibody Ranibizumab
DIQLTQSPSSLSASVGDRVTITCSASQDISNYLNWYQQKPGKAPKVLIYFTSSLHSGVPSRFSGSGSGTDFTLTISSLQPEDFATYYCQQYSTVPWTFGQGTKVEIKRTVAAPSVFIFPPSDEQLKSGTASVVCLLNNFYPREAKVQWKVDNALQSGNSQESVTEQDSKDSTYSLSSTLTLSKADYEKHKVYACEVTHQGLSSPVTKSFNRGEC

SEQ ID NO: 161 - protein, 446 aa, synthetic construct
  REGION 1..446: note = Heavy chain of anti-VEGF antibody Ramucirumab
EVQLVQSGGGLVKPGGSLRLSCAASGFTFSSYSMNWVRQAPGKGLEWVSSISSSSSYIYYADSVKGRFTISRDNAKNSLYLQMNSLRAEDTAVYYCARVTDAFDIWGQGTMVTVSSASTKGPSVFPLAPSSKSTSGGTAALGCLVKDYFPEPVTVSWNSGALTSGVHTFPAVLQSSGLYSLSSVVTVPSSSLGTQTYICNVNHKPSNTKVDKKVEPKSCDKTHTCPPCPAPELLGGPSVFLFPPKPKDTLMISRTPEVTCVVVDVSHEDPEVKFNWYVDGVEVHNAKTKPREEQYNSTYRVVSVLTVLHQDWLNGKEYKCKVSNKALPAPIEKTISKAKGQPREPQVYTLPPSREEMTKNQVSLTCLVKGFYPSDIAVEWESNGQPENNYKTTPPVLDSDGSFFLYSKLTVDKSRWQQGNVFSCSVMHEALHNHYTQKSLSLSPGK

SEQ ID NO: 162 - protein, 214 aa, synthetic construct
  REGION 1..214: note = Light chain of anti-VEGF antibody Ramucirumab
DIQMTQSPSSVSASIGDRVTITCRASQGIDNWLGWYQQKPGKAPKLLIYDASNLDTGVPSRFSGSGSGTYFTLTISSLQAEDFAVYFCQQAKAFPPTFGGGTKVDIKGTVAAPSVFIFPPSDEQLKSGTASVVCLLNNFYPREAKVQWKVDNALQSGNSQESVTEQDSKDSTYSLSSTLTLSKADYEKHKVYACEVTHQGLSSPVTKSFNRGEC

SEQ ID NO: 163 - protein, 453 aa, synthetic construct
  REGION 1..453: note = Heavy chain of anti-VEGF antibody Faricimab
EVQLVESGGGLVQPGGSLRLSCAASGYDFTHYGMNWVRQAPGKGLEWVGWINTYTGEPTYAADFKRRFTFSLDTSKSTAYLQMNSLRAEDTAVYYCAKYPYYYGTSHWYFDVWGQGTLVTVSSASTKGPSVFPLAPSSKSTSGGTAALGCLVKDYFPEPVTVSWNSGALTSGVHTFPAVLQSSGLYSLSSVVTVPSSSLGTQTYICNVNHKPSNTKVDKKVEPKSCDKTHTCPPCPAPEAAGGPSVFLFPPKPKDTLMASRTPEVTCVVVDVSHEDPEVKFNWYVDGVEVHNAKTKPREEQYNSTYRVVSVLTVLAQDWLNGKEYKCKVSNKALGAPIEKTISKAKGQPREPQVYTLPPCRDELTKNQVSLWCLVKGFYPSDIAVEWESNGQPENNYKTTPPVLDSDGSFFLYSKLTVDKSRWQQGNVFSCSVMHEALHNAYTQKSLSLSPGK

SEQ ID NO: 164 - protein, 214 aa, synthetic construct; identical to SEQ ID NO: 160
  REGION 1..214: note = Light chain of anti-VEGF antibody Faricimab

SEQ ID NO: 165 - protein, 453 aa, synthetic construct
  REGION 1..453: note = Heavy chain of anti-VEGF antibody KSI-301
EVQLVESGGGLVQPGGSLRLSCAASGYDFTHYGMNWVRQAPGKGLEWVGWINTYTGEPTYAADFKRRFTFSLDTSKSTAYLQMNSLRAEDTAVYYCAKYPYYYGTSHWYFDVWGQGTLVTVSSASTKGPSVFPLAPSSKSTSGGTAALGCLVKDYFPEPVTVSWNSGALTSGVHTFPAVLQSSGLYSLSSVVTVPSSSLGTQTYICNVNHKPSNTKVDKKVEPKSCDKTHTCPPCPAPEAAGAPSVFLFPPKPKDTLMISRTPEVTCVVVDVSHEDPEVKFNWYVDGVEVHNAKTKPREEQYNSTYRVVSVLTVLHQDWLNGKEYKCKVSNKALPAPIEKTISKAKGQPREPQVYTLPPSREEMTKNQVSLTCLVKGFYPSDIAVEWESNGQPENNYKTTPPVLDSDGSFFLYSKLTVDKSRWQQGNVFSCSVMHEALHNHYTQKSLSCSPGK

SEQ ID NO: 166 - protein, 214 aa, synthetic construct; identical to SEQ ID NO: 160
  REGION 1..214: note = Light chain of anti-VEGF antibody KSI-301

SEQ ID NO: 167 - protein, 453 aa, synthetic construct
  REGION 1..453: note = Heavy chain of anti-VEGF antibody Vanucizumab
EVQLVESGGGLVQPGGSLRLSCAASGYTFTNYGMNWVRQAPGKGLEWVGWINTYTGEPTYAADFKRRFTFSLDTSKSTAYLQMNSLRAEDTAVYYCAKYPHYYGSSHWYFDVWGQGTLVTVSSASTKGPSVFPLAPSSKSTSGGTAALGCLVKDYFPEPVTVSWNSGALTSGVHTFPAVLQSSGLYSLSSVVTVPSSSLGTQTYICNVNHKPSNTKVDKKVEPKSCDKTHTCPPCPAPELLGGPSVFLFPPKPKDTLMISRTPEVTCVVVDVSHEDPEVKFNWYVDGVEVHNAKTKPREEQYNSTYRVVSVLTVLHQDWLNGKEYKCKVSNKALPAPIEKTISKAKGQPREPQVYTLPPCRDELTKNQVSLWCLVKGFYPSDIAVEWESNGQPENNYKTTPPVLDSDGSFFLYSKLTVDKSRWQQGNVFSCSVMHEALHNHYTQKSLSLSPGK

SEQ ID NO: 168 - protein, 214 aa, synthetic construct; identical to SEQ ID NO: 158
  REGION 1..214: note = Light chain of anti-VEGF antibody Vanucizumab

SEQ ID NO: 169 - protein, 453 aa, synthetic construct
  REGION 1..453: note = Heavy chain of BAT-5906
EVQLVESGGGLVQPGGSLRLSCAASGYDFTHYGMNWVRQAPGKGLEWVGWINTYTGEPTYAADFKRRFTFSLDTSKSTAYLQMNSLRAEDTAVYYCAKYPYYYGTSHWYFDVWGQGTLVTVSSASTKGPSVFPLAPSSKSTSGGTAALGCLVKDYFPEPVTVSWNSGALTSGVHTFPAVLQSSGLYSLSSVVTVPSSSLGTQTYICNVNHKPSNTKVDKKVEPKSCDKTHTCPPCPAPELLGGPSVFLFPPKPKDTLMISRTPEVTCVVVDVSHEDPEVKFNWYVDGVEVHNAKTKPREEQYNSTYRVVSVLTVLHQDWLNGKEYKCKVSNKALPAPIEKTISKAKGQPREPQVYTLPPSREEMTKNQVSLTCLVKGFYPSDIAVEWESNGQPENNYKTTPPVLDSDGSFFLYSKLTVDKSRWQQGNVFSCSVMHEALHNHYTQKSLSLSPGK

SEQ ID NO: 170 - protein, 214 aa, synthetic construct; identical to SEQ ID NO: 160
  REGION 1..214: note = Light chain of BAT-5906

SEQ ID NO: 171 - protein, 447 aa, synthetic construct
  REGION 1..447: note = Heavy chain of Navicixizumab
QVQLVQSGAEVKKPGASVKVSCKASGYTFTNYWMHWVRQAPGQGLEWMGDINPSNGRTSYKEKFKRRVTLSVDKSSSTAYMELSSLRSEDTAVYFCTIHYDDKYYPLMDYWGQGTLVTVSSASTKGPSVFPLAPCSRSTSESTAALGCLVKDYFPEPVTVSWNSGALTSGVHTFPAVLQSSGLYSLSSVVTVPSSNFGTQTYTCNVDHKPSNTKVDKTVERKCCVECPPCPAPPVAGPSVFLFPPKPKDTLMISRTPEVTCVVVDVSHEDPEVQFNWYVDGVEVHNAKTKPREEQFNSTFRVVSVLTVVHQDWLNGKEYKCKVSNKGLPAPIEKTISKTKGQPREPQVYTLPPSREKMTKNQVSLTCLVKGFYPSDIAVEWESNGQPENNYKTTPPMLKSDGSFFLYSKLTVDKSRWQQGNVFSCSVMHEALHNHYTQKSLSLSPGK

SEQ ID NO: 172 - protein, 218 aa, synthetic construct
  REGION 1..218: note = Light chain of Navicixizumab
DIVMTQSPDSLAVSLGERATISCRASESVDNYGISFMKWFQQKPGQPPKLLIYAASNQGSGVPDRFSGSGSGTDFTLTISSLQAEDVAVYYCQQSKEVPWTFGGGTKVEIKRTVAAPSVFIFPPSDEQLKSGTASVVCLLNNFYPREAKVQWKVDNALQSGNSQESVTEQDSKDSTYSLSSTLTLSKADYEKHKVYACEVTHQGLSSPVTKSFNRGEC

SEQ ID NO: 173 - protein, 577 aa, synthetic construct
  REGION 1..577: note = Heavy chain of Dilpacimab
EVQLVESGGGLVQPGGSLRLSCAASGFTFSNFPMAWVRQAPGKGLEWVATISSSDGTTYYRDSVKGRFTISRDNAKNSLYLQMNSLRAEDTAVYYCARGYYNSPFAYWGQGTLVTVSSASTKGPEVQLVESGGGLVQPGGSLRLSCAASGYTFTNYGMNWVRQAPGKGLEWVGWINTYTGEPTYAADFKRRFTFSLDTSKSTAYLQMNSLRAEDTAVYYCAKYPHYYGSSHWYFDVWGQGTLVTVSSASTKGPSVFPLAPSSKSTSGGTAALGCLVKDYFPEPVTVSWNSGALTSGVHTFPAVLQSSGLYSLSSVVTVPSSSLGTQTYICNVNHKPSNTKVDKKVEPKSCDKTHTCPPCPAPEAAGGPSVFLFPPKPKDTLMISRTPEVTCVVVDVSHEDPEVKFNWYVDGVEVHNAKTKPREEQYNSTYRVVSVLTVLHQDWLNGKEYKCKVSNKALPAPIEKTISKAKGQPREPQVYTLPPSREEMTKNQVSLTCLVKGFYPSDIAVEWESNGQPENNYKTTPPVLDSDGSFFLYSKLTVDKSRWQQGNVFSCSVMHEALHNHYTQKSLSLSPGK

SEQ ID NO: 174 - protein, 334 aa, synthetic construct
  REGION 1..334: note = Light chain of Dilpacimab
DIQMTQSPSSLSASVGDRVTITCRASEDIYSNLAWYQQKPGKAPKLLIYDTNNLADGVPSRFSGSGSGTDFTLTISSLQPEDFATYYCQQYNNYPPTFGQGTKLEIKRTVAAPSVFIFPPDIQMTQSPSSLSASVGDRVTITCSASQDISNYLNWYQQKPGKAPKVLIYFTSSLHSGVPSRFSGSGSGTDFTLTISSLQPEDFATYYCQQYSTVPWTFGQGTKVEIKRTVAAPSVFIFPPSDEQLKSGTASVVCLLNNFYPREAKVQWKVDNALQSGNSQESVTEQDSKDSTYSLSSTLTLSKADYEKHKVYACEVTHQGLSSPVTKSFNRGEC

SEQ ID NO: 175 - protein, 116 aa, synthetic construct
  REGION 1..116: note = Heavy chain variable regions of hPV-19
DVQLVQSGVEVKNPGASVKVSCRASGYSFTNSGINWVKQAPGKGLKWMGWINTYTGEPTYADDFKGRFAFSLETSASSAYLQINNLKNEDTATYFCARFGDGYYWFFDVWGAGTTV

SEQ ID NO: 176 - protein, 113 aa, synthetic construct
  REGION 1..113: note = Light chain variable regions of hPV-19
DIVMTQSPDSLAVSLGERATINCKSSQSLLNSRTRKNFLAWYQQKPGQSPKLLIYWASTRESGVPDRFTGSGSGTDFTLTISSVQAEDLAVYYCKQSYNLYTFGGGTNLEIKR

SEQ ID NO: 177 - protein, 126 aa, synthetic construct
  REGION 1..126: note = Heavy chain variable regions of AT-001
QVQLVQSGAEVKKPGASVKVSCKASGGTFSSYAISWVRQAPGQGLEWMGGFDPEDGETIYAQKFQGRVTMTEDTSTDTAYMELSSLRSEDTAVYYCATGRSMVRGVIIPFNGMDVWGQGTTVTVSS

SEQ ID NO: 178 - protein, 107 aa, synthetic construct
  REGION 1..107: note = Light chain variable regions of AT-001
DIRMTQSPSSLSASVGDRVTITCRASQSISSYLNWYQQKPGKAPKLLIYAASSLQSGVPSRFSGSGSGTDFTLTISSLQPEDFATYYCQQSYSTPLTFGGGTKVEIK

SEQ ID NO: 179 - protein, 11 aa, synthetic construct
  REGION 1..11: note = CDR1 of Brolucizumab
QASEIIHSWLA

SEQ ID NO: 180 - protein, 7 aa, synthetic construct
  REGION 1..7: note = CDR2 of Brolucizumab
LASTLAS

SEQ ID NO: 181 - protein, 12 aa, synthetic construct
  REGION 1..12: note = CDR3 of Brolucizumab
QNVYLASTNGAN

SEQ ID NO: 182 - protein, 11 aa, synthetic construct
  REGION 1..11: note = CDR4 of Brolucizumab
GFSLTDYYYMT

SEQ ID NO: 183 - protein, 16 aa, synthetic construct
  REGION 1..16: note = CDR5 of Brolucizumab
FIDPDDDPYYATWAKG

SEQ ID NO: 184 - protein, 11 aa, synthetic construct
  REGION 1..11: note = CDR6 of Brolucizumab
GDHNSGWGLDI

SEQ ID NO: 185 - protein, 252 aa, synthetic construct
  REGION 1..252: note = scFv of anti-VEGF antibody Brolucizumab (VL-linker-VL)
MEIVMTQSPSTLSASVGDRVIITCQASEIIHSWLAWYQQKPGKAPKLLIYLASTLASGVPSRFSGSGSGAEFTLTISSLQPDDFATYYCQNVYLASTNGANFGQGTKLTVLGGGGGSGGGGSGGGGSGGGGSEVQLVESGGGLVQPGGSLRLSCTASGFSLTDYYYMTWVRQAPGKGLEWVGFIDPDDDPYYATWAKGRFTISRDNSKNTLYLQMNSLRAEDTAVYYCAGGDHNSGWGLDIWGQGTLVTVSS

SEQ ID NO: 186 - protein, 11 aa, synthetic construct
  REGION 1..11: note = HC-CDR1 of HuMab G6-31
SASQDISNYLN

SEQ ID NO: 187 - protein, 16 aa, synthetic construct
  REGION 1..16: note = HC-CDR2 of HuMab G6-31
GITPAGGYTYYADSVK

SEQ ID NO: 188 - protein, 5 aa, synthetic construct
  REGION 1..5: note = HC-CDR3 of HuMab G6-31
DYWIH

SEQ ID NO: 189 - protein, 9 aa, synthetic construct
  REGION 1..9: note = LC-CDR1 of HuMab G6-31
QQGYGNPFT

SEQ ID NO: 190 - protein, 7 aa, synthetic construct
  REGION 1..7: note = LC-CDR2 of HuMab G6-31
SASFLYS

SEQ ID NO: 191 - protein, 11 aa, synthetic construct
  REGION 1..11: note = LC-CDR3 of HuMab G6-31
RASQDVSTAVA

SEQ ID NO: 192 - protein, 12 aa, synthetic construct
  REGION 1..12: note = HC-CDR1 of B20-4.1
WGHSTSPWAMDY

SEQ ID NO: 193 - protein, 16 aa, synthetic construct
  REGION 1..16: note = HC-CDR2 of B20-4.1
AIWPFGGYTHYADSVK

SEQ ID NO: 194 - protein, 8 aa, synthetic construct
  REGION 1..8: note = HC-CDR3 of B20-4.1
FSINGSWI

SEQ ID NO: 195 - protein, 9 aa, synthetic construct
  REGION 1..9: note = LC-CDR1 of B20-4.1
QQSNTSPLT

SEQ ID NO: 196 - protein, 8 aa, synthetic construct
  REGION 1..8: note = LC-CDR2 of B20-4.1
YAASNLAS

SEQ ID NO: 197 - protein, 11 aa, synthetic construct
  REGION 1..11: note = LC-CDR3 of B20-4.1
RASQVIRRSLA